European Patent Application EP 4 707 387 A2, published March 11, 2026. Title: Attenuated Dengue Viruses. Applicant: Codagenix Inc. Application EP. The sequence listing filed with the application follows.

SEQUENCE LISTING (12 sequences)

SEQ ID NO: 1 - DNA, 10735 bp, Dengue virus
  source 1..10735: mol_type = genomic DNA
agttgttagtctacgtggaccgacaagaacagtttcgaatcggaagcttgcttaacgtagttctaacagttttttattagagagcagatctctgatgaacaaccaacggaaaaagacggctcgaccgtctttcaatatgctgaaacgcgcgagaaaccgcgtgtcaactgtttcacagttggcgaagagattctcaaaaggattgctctcaggccaaggacccatgaaattggtgatggctttcatagcattcctaagatttctagccatacccccaacagcaggaattttggctagatggggttcattcaagaagagtggagcgatcaaagtgctacggggtttcaagaaagaaatctcaaacatgttgaatataatgaatagaaggaaaagatctgtgaccatgctccttatgctgatgcctacagccttggcgttccatttgactacacgagggggagagccgcacatgatagtcagcaagcaggaaagaggaaagtcactcttgtttaagacctcagcaggtgtcaacatgtgcacccttatagcgatggatttgggagagttatgtgaggacacaatgacttacaaatgccctcgaatcactgaaactgaaccagatgacgttgattgttggtgtaatgccacagacacatgggtgacctatggaacatgttcccaaactggcgagcaccgacgagacaaacgttccgtcgcactggccccacacgtgggacttggtttggaaacaagaaccgaaacgtggatgtcctctgaaggcgcttggaaacagatacaaagagtggagacttgggccctgagacacccaggattcacggtgatagccctttttctagcacatgccataggaacatccatcacccagaaagggattattttcattttgttaatgctggtaacaccatccatggccatgcgatgcgtgggaataggcagcagggacttcgtggaaggactgtcaggagcaacttgggtagatgtggtactggaacatggaagttgcgtcaccaccatggcaaaagacaaaccaacattggacattgaactcttgaagacggaagtcacaaaccctgccgtcctgcgcaaactgtgcattgaagctaaaatatcaaacaccaccaccgactcaagatgtccaacacaaggagaagccacactagtggaagaacaagacgcgaactttgtgtgtcgacgaacgtttgtggacagaggctggggcaatggctgtggcctcttcggaaaaggaagcctaataacgtgtgcaaagttcaagtgtgtgacaaaactggaaggaaagatagttcaatatgagaacttgaaatattcagtaatagtcaccgttcacaccggagaccagcatcaagtgggaaatgaaagcacagaacatgggacaactgcaactataacacctcaagctcctacgacggaaatacagctgaccgactacggagctcttacattggattgttcacctagaacaggactagactttaatgaaatggtgttgttgacaatgaaagaaaaatcatggctagtccacaaacaatggtttttagacctaccactgccttggacctcgggagcttcaacatcacaagagacttggaacagacaagatttgctggtgacatttaagacagctcatgcaaagaagcaggaagtagtcgtactaggatcacaagaaggagcaatgcacactgcgttgaccggagcgacagaaatccaaacgtctggaacgacaacaatttttgcaggacacttgaaatgcagactaaagatggacaaactgactctaaaagggatgtcatatgtgatgtgcacaggctcattcaagctagagaaagaagtggctgagacccagcatggaaccgttctagtgcagattaaatacgaaggaacagatgcaccatgcaagatccctttttcgacccaagatgaaaaaggagtaacccagaatgggagattgataacagctaaccccatagttactgacaaagaaaaaccagtcaacattgaggcagaaccgccctttggtgagagttacatcgtaataggagcaggtgaaaaagctttgaaactaagctggttcaagaaaggaagcagcatagggaaaatgtttgaggcaactgccagaggagcacgaaggatggccatactgggagacaccgcatgggactttggttctataggaggagtgttcacgtctgttggaaaattagtacaccagatttttggaactgcatatggagttttgttcagcggtgtttcctggaccatgaaaataggaataggggttctgctgacatggctgggattaaactcaaggagcacgtccctttcgatgacgtgcattgcagttggcctagtaacactatacctaggagtcatggttcaggcggattcaggatgtgtaattaattggaaaggtagagaactcaagtgtggaagtggcatttttgtcaccaatgaagttcacacttggacagagcaatacaaatttcaagctgactcccctaagagactatcagcagccatcgggaaggcatgggaggagggtgtgtgtggaattcgatcagcaactcgtctcgagaacatcatgtggaagcaaatatcaaatgaactgaatcacatcttacttgaaaatgatatgaaattcacagtggttgtaggagatgttgctgggatcttggctcaaggaaagaaaatgattaggccacaacccatggaatacaaatactcgtggaaaagctggggaaaggctaaaatcataggggcagatgtacagaacaccaccttcatcatcgatggcccaaacaccccagaatgccctgatgaccaaagagcatggaacatttgggaagttgaggactatggatttggaattttcacgacaaacatatggctgaaattgcgtgattcctacacccaagtgtgtgaccaccggctaatgtcagctgccatcaaggacagcaaggcagttcacgctgacatggggtactggatagaaagtgaaaagaacgagacctggaagctggcaagagcctcattcatagaagttaaaacatgtatctggccaaaatcccacactctatggagcaatggagttctggaaagtgaaatgataattccaaagatctatggaggaccaatatctcagcacaactacagaccaggatattttacacaagcagcagggccgtggcacctaggcaagttggaactggattttgatttgtgtgagggtaccacagttgttgtggatgaacattgtggaaatcgaggaccatctcttaggaccacaacagtcacaggaaagataattcatgaatggtgttgcagatcttgcacgctaccacccttacgtttcagaggagaagatgggtgctggtacggtatggaaatcagaccagtcaaggaaaaggaagaaaatctagtcaaatcaatggtctctgcagggtcaggggaagtggacagcttttcactaggactgctatgcatatcaataatgatcgaggaggtgatgagatccagatggagtagaagaatgctgatgactggaacactggctgtgttcttccttctcataatgggacaattgacatggaacgatctgatcagattatgcatcatggttggagccaacgcttccgacaggatggggatgggaacgacgtacctagccctgatggccacttttaaaatgagaccgatgttcgctgtagggctattatttcgcagactaacatccagagaagttcttcttctaacaattggattgagtctagtggcatctgtggagttaccaaattccttggaggagctgggggatggacttgcaatgggcattatgattttaaaattattgactgactttcaatcacatcagctgtgggctaccttgctgtccttgacatttatcaaaacaacgttttccttgcactacgcatggaagacaatggctatggtactgtcaattgtatctctcttccctttatgcctgtccacgacctcccaaaaaacaacatggcttccggtgctattgggatcccttggatgcaaaccactaaccatgtttcttatagcagaaaacaaaatctggggaaggagaagttggcccctcaatgaaggaatcatggctgttggaatagtcagcatcctactaagttcactcctcaaaaatgatgtaccgctagctgggccactaatagctggaggcatgctaatagcatgttatgttatatctggaagctcagccgacctatcattagagaaagcggctgaggtctcctgggaagaagaagcagaacactctggtgcctcacacaacatattagtggaagtccaagatgatggaaccatgaagataaaggatgaagagagagatgacacgctaaccattctccttaaagcaactctgttagcagtttcaggggtgtacccattatcaataccagcgacccttttcgtgtggtacttttggcagaaaaagaaacagagatctggagtgttatgggacacacccagccctccagaagtggaaagagcagttcttgatgatggtatctatagaattatgcagagaggactgttgggcaggtcccaagtaggggtaggagttttccaagaaaacgtgttccacacaatgtggcatgtcaccaggggagctgtactcatgtatcaagggaagagattggaaccgagctgggccagtgtcaaaaaagacctgatctcatatggaggaggttggaggcttcaaggatcctggaacacaggagaagaagtgcaggtgattgctgttgaaccagggaaaaaccccaaaaatgtacaaacagcgccgggcacctttaagacccctgaaggtgaagttggagccattgccctagactttaaacctggcacatctggatctcccatcgtgaacagagaaggaaaaatagtaggtctttatggaaatggagtagtgacaacaagtggaacctacgtcagtgccatagctcaagccaaagcatcacaagaagggcccctaccagagattgaagacgaggtgtttaggaaaagaaacttaacaataatggacctacatccaggatcggggaaaacaagaagatatcttccagccatagtccgtgaggccataaaaaggaagctgcgcacactaatcctggctcccacaagggttgtcgcttccgaaatggcagaggcgctcaagggaatgccaataaggtaccaaacaacagcagtgaagagtgaacatacaggaaaagagatagttgacctcatgtgtcacgccactttcaccatgcgcctcctgtctcccgtaagagttcccaattacaacatgatcatcatggatgaagcacatttcaccgatccatccagtatagcggccagagggtacatctcaacccgagtgggcatgggtgaagcagctgcaatcttcatgacagccactcccccaggatcagtggaggcctttccacagagcaacgcagttatccaagatgaggaaagagacattcctgagagatcatggaactcaggctatgagtggatcactgacttcccaggtaaaacagtttggtttgttccaagcattaaatcaggaaatgacattgccaactgcttaagaaagaatgggaaacgggtgattcaattgagcaggaaaacctttgatacagagtaccaaaaaacaaaaaacaacgactgggactacgtcgtcacaacagacatctccgaaatgggagcaaatttccgagccgacagggtgatagacccaagacggtgtctgaaaccggtaatactaaaagatggtccagagcgtgtcattttagcaggaccaatgccagtgactgtggccagtgccgctcagaggagaggaagaattggaaggaaccacaataaggaaggtgatcagtacatctacatgggacagcctttaaacaacgatgaagatcacgctcactggacagaagcaaaaatgctccttgataatataaacacaccagaagggattatcccagccctctttgagccagagagagaaaagagtgcagcaatagacggggaatacagactgcggggtgaagcaaggaaaacgtttgtggagctcatgagaagaggagatctacctgtctggctatcctacaaagttgcctcagaaggcttccagtactctgacagaagatggtgctttgacggggaaaggaacaaccaggtgttggaggagaacatggacgtggagatctggacaaaagaaggagaaagaaagaaactacgaccccgctggctggatgccagaacatactcagacccactagccctgcgcgagtttaaagagtttgcagcagggagaagaagcgtctcaggtgatttaatattagaaatagggaagcttccacaacacttgacgcaaagggcccagaatgccctggacaacctggttatgttgcacaactccgaacaaggaggcagagcctatagacatgcaatggaagaactgccagacaccatagaaacgttgatgctcctagctttgatagctgtgttaactggtggagtgacactgttcttcctatcaggaaggggcctagggaaaacatctatcggcctactctgcgtaatggcttcaagcgtactgctatggatggccagtgtggagccccattggatagcggcctccatcatactggagttcttcctgatggtgctgcttattccagagccagacagacaacgcactccgcaggacaaccagctggcatatgtggtgataggtttgttattcatgatactgacagtagcagccaatgagatgggactgctggaaaccacaaagaaagacttagggattggccatgtggctgttgaaaatcaccaccatgccgcaatgctggacgtagacttacatccagcttcagcctggaccctctatgcagtggccacaacaattatcactcccatgatgaggcacacaatcgaaaacacaacggcaaacatttccctgacagccattgcaaaccaggcagctatattgatgggacttgacaaaggatggccaatatcgaagatggacataggagttccacttctcgccttggggtgctattcccaggtgaatccactgacgctgacagcggcggtattgatgctagtggctcattacgccataattggacctggactgcaagcaaaagctactagagaagctcaaaaaaggacagcggccggaataatgaaaaatccaaccgttgatggaattgttgcaatagatttggaccctgtggtttatgatgcaaaatttgaaaaacaactaggccaaataatgttgttgatactatgcacatcacagatcctcttgatgcggactacatgggccttgtgcgagtccatcacactggccactggacctctgaccacgctttgggagggatctccaggaaaattttggaacaccacgatagcggtttccatggcaaacattttcagaggaagttatctagcaggagcaggtctggccttctcattaatgaaatctctaggaggaggtaggagaggcacgggagcccaaggggaaacactgggagagaaatggaaaagacagctgaaccaactgagcaagtcagaatttaacacctataaaaggagtgggattatggaagtggacagatccgaagccaaagagggattgaaaagaggagaaacaaccaaacatgcagtgtcgagaggaaccgctaaactgaggtggttcgtggagaggaaccttgtgaaaccagaagggaaagtcatagacctcggttgtggaagaggtggctggtcatactattgcgctgggctgaagaaagtcacagaagtgaaggggtatacaaaaggaggacctggacatgaggaaccaatcccaatggcgacctatggatggaacctagtaaagctgcactctgggaaagacgtattttttataccacctgagaaatgtgacacccttttgtgtgatattggtgagtcctctccaaacccaactatagaggaaggaagaacgctacgcgtcctaaagatggtggaaccatggctcagaggaaaccaattttgcataaaaattctgaatccctacatgccaagtgtggtggaaactctggagcaaatgcaaagaaaacatggaggaatgctagtgcgaaatccactttcaagaaattctactcatgaaatgtattgggtttcatgtggaacaggaaacattgtgtcagcagtaaacatgacatctagaatgttgctaaatcgattcacaatggctcacaggaaaccaacatatgaaagagacgtggacctaggcgccggaacaagacatgtggcagtggaaccagaggtagccaacctagatatcattggccagaggatagagaacataaaacatgaacataagtcaacatggcattatgatgaggacaatccatataaaacatgggcctatcatggatcatatgaggtcaagccatcaggatcagcctcatccatggtcaatggcgtggtgaaactgctcaccaaaccatgggatgtcatccctatggtcacacaaatagccatgactgacactacaccctttggacaacagagggtgtttaaagagaaagttgacacacgcacaccaaaagcaaaacggggcacagcacaaatcatggaggtgacagccaagtggttatggggttttctttctagaaacaagaaaccaagaatttgcacaagagaggagttcacaagaaaagttaggtcaaacgcagccattggagcagtgttcgttgatgaaaatcaatggaactcagcaaaagaagcagtggaagatgagcggttctgggaccttgtgcatagagagagggagcttcacaaacagggaaaatgtgctacgtgtgtttacaacatgatggggaagagagagaaaaagctaggagagttcggaaaggcaaaaggaagtcgtgcaatatggtacatgtggttgggagcacgctttctagagttcgaagctcttggtttcatgaacgaagatcactggttcagcagagagaattcactcagcggagtggaaggagaaggactccacaaacttggatatatactcagagacatatcaaagattccagggggaaacatgtatgcagatgacacagccggatgggatacaaggataacagaggatgaccttcagaatgaggccagaattactgacatcatggaacccgaacatgccctcctggctaagtcaatcttcaagttaacctaccaaaataaggtggtaagggtacagagaccagcaaaaaatggaaccgtgatggatgtcatatccagacgtgaccagagaggaagtggtcaggtcggaacttatggcttaaacactttcaccaacatggaagcccagctgataagacaaatggagtctgagggaatcttttcacccagcgaattagagaccccaaatttagccgagagagttctcgactggctggaaaaatatggcgtcgaaaggctgaaaagaatggcaatcagcggagatgactgcgtagtgaaaccaattgatgataggtttgcaacagccttgacagctctgaatgatatgggaaaagtaagaaaagatataccacaatgggaaccttcaaaaggatggaatgattggcaacaagtgcctttttgttcacaccacttccaccagctgattatgaaggatgggagggaaatagtggtgccatgccgcaaccaagatgaacttgtgggtagggctagagtatcacaaggtgctggatggagcctgagagaaactgcatgcctaggcaagtcatatgcacaaatgtggcagctgatgtacttccacaggagagacctgagactagccgctaatgctatctgttcagccgttccagttgattggatcccaaccagccgtaccacctggtcgatccatgcccatcaccaatggatgacaacagaagacatgctgtcagtgtggaatagggtttggatagaggaaaacccatggatggaggacaaaacccacatatccagttggggagatgttccatatttaggaaaaagggaagaccaatggtgtggatccctgataggcttaacagcaagggccacctgggccaccaacatacaagtggccataaaccaagtgagaagactaattgggaatgagaattatctagattacatgacatcaatgaagagattcaagaacgagagtgatcccgaaggggcactctggtgagtcaacacatttacaaaataaaggaaaataagaaatcaaacaaggcaagaagtcaggccggattaagccatagtacggtaagagctatgctgcctgtgagccccgtctaaggacgtaaaatgaagtcaggccgaaagccacggcttgagcaaaccgtgctgcctgtagctccatcgtggggatgtaaaaacctgggaggctgcaacccatggaagctgtacgcatggggtagcagactagtggttagaggagacccctcccgaaacataacgcagcagcggggcccaacaccaggggaagctgtaccctggtggtaaggactagaggttagaggagaccccccgcataacaataaacagcatattgacgctgggagagaccagagatcctgctgtctctacagcatcattccaggcacagaacgccagaaaatggaatggtgctgttgaatcaacaggttct

SEQ ID NO: 2 - DNA, 10735 bp, Dengue virus
  source 1..10735: mol_type = genomic DNA
agttgttagtctacgtggaccgacaagaacagtttcgaatcggaagcttgcttaacgtagttctaacagttttttattagagagcagatctctgatgaacaaccaacggaaaaagacggctcgaccgtctttcaatatgctgaaacgcgcgagaaaccgcgtgtcaactgtttcacagttggcgaagagattctcaaaaggattgctctcaggccaaggacccatgaaattggtgatggctttcatagcattcctaagatttctagccatacccccaacagcaggaattttggctagatggggttcattcaagaagagtggagcgatcaaagtgctacggggtttcaagaaagaaatctcaaacatgttgaatataatgaatagaaggaaaagatctgtgaccatgctccttatgctgatgcctacagccttggcgttccatttgactacacgagggggagagccgcacatgatagtcagcaagcaggaaagaggaaagtcactcttgtttaagacctcagcaggtgtcaacatgtgcacccttatagcgatggatttgggagagttatgtgaggacacaatgacttacaaatgccctcgaatcactgaaactgaaccagatgacgttgattgttggtgtaatgccacagacacatgggtgacctatggaacatgttcccaaactggcgagcaccgacgagacaaacgttccgtcgcactggccccacacgtgggacttggtttggaaacaagaaccgaaacgtggatgtcctctgaaggcgcttggaaacagatacaaagagtggagacttgggccctgagacacccaggattcacggtgatagccctttttctagcacatgccataggaacatccatcacccagaaagggattattttcattttgttaatgctggtaacaccatccatggccatgcgatgcgtagggatagggtcacgcgatttcgtcgaaggactatccggagcgacatgggtcgacgtcgtactcgaacacggatcatgcgttacgactatggctaaagacaaacctacactagacatagagttactgaaaaccgaagttacgaatcccgccgtactgcgaaaattgtgtatcgaagcgaaaattagcaatacgactacagactctaggtgtcctacacaaggcgaagcgacattggtcgaagaacaggacgctaacttcgtatgtagacgaacattcgtcgatagggggtggggaaacggatgcggattgttcggtaaaggatcactgattacatgcgcaaagttcaaatgcgttacgaaactggaaggtaaaatagtgcaatacgaaaacctaaagtatagcgtaatcgttacagtgcataccggagaccaacatcaggtcggaaacgaatcaaccgaacacggaacaaccgcaacaattacaccacaggcacctacaaccgaaattcaactaaccgattacggagctcttacactagattgctcacctagaaccggattggactttaacgaaatggtactgttgactatgaaggagaaatcatggttagtgcataaacaatggtttctagacctaccactaccatggactagcggagcgagtacgtcacaggaaacatggaatagacaggacctattggtgacatttaagaccgcacacgctaagaagcaggaagtcgtagtgttagggtcacaagagggagcaatgcataccgcactaaccggagcaaccgaaatacagactagcggaactacaacgatttttgccggtcacctgaaatgtagactgaagatggacaaactgacacttaaaggaatgtcatacgttatgtgtacgggatcctttaagctcgaaaaagaggttgccgaaacgcaacacggaacagtgctagtgcaaattaaatatgagggaaccgacgcaccatgtaagataccgtttagtacgcaagacgaaaagggcgttacgcaaaacggaagactgattaccgctaaccctatcgttacagacaaagagaaacccgttaacatagaggccgaaccaccttttggcgaatcatatatagtgataggcgcaggcgaaaaagcactaaagctgtcatggttcaaaaaaggatctagcatagggaagatgttcgaagcaaccgctaggggagctagacgaatggcaatactgggagataccgcatgggacttcggatcgatagggggagtgtttactagcgtaggtaagttggtgcatcagatattcggaaccgcatacggagtgttgtttagcggagtgtcatggactatgaagatagggataggagtgctattgacatggctcggactgaattcgagatcgactagcctatctatgacatgcatagccgtcggactggttacactgtatctaggcgtaatggtgcaagcagattcaggatgtgtaattaattggaaaggtagagaactcaagtgtggaagtggcatttttgtcaccaatgaagttcacacttggacagagcaatacaaatttcaagctgactcccctaagagactatcagcagccatcgggaaggcatgggaggagggtgtgtgtggaattcgatcagcaactcgtctcgagaacatcatgtggaagcaaatatcaaatgaactgaatcacatcttacttgaaaatgatatgaaattcacagtggttgtaggagatgttgctgggatcttggctcaaggaaagaaaatgattaggccacaacccatggaatacaaatactcgtggaaaagctggggaaaggctaaaatcataggggcagatgtacagaacaccaccttcatcatcgatggcccaaacaccccagaatgccctgatgaccaaagagcatggaacatttgggaagttgaggactatggatttggaattttcacgacaaacatatggctgaaattgcgtgattcctacacccaagtgtgtgaccaccggctaatgtcagctgccatcaaggacagcaaggcagttcacgctgacatggggtactggatagaaagtgaaaagaacgagacctggaagctggcaagagcctcattcatagaagttaaaacatgtatctggccaaaatcccacactctatggagcaatggagttctggaaagtgaaatgataattccaaagatctatggaggaccaatatctcagcacaactacagaccaggatattttacacaagcagcagggccgtggcacctaggcaagttggaactggattttgatttgtgtgagggtaccacagttgttgtggatgaacattgtggaaatcgaggaccatctcttaggaccacaacagtcacaggaaagataattcatgaatggtgttgcagatcttgcacgctaccacccttacgtttcagaggagaagatgggtgctggtacggtatggaaatcagaccagtcaaggaaaaggaagaaaatctagtcaaatcaatggtctctgcagggtcaggggaagtggacagcttttcactaggactgctatgcatatcaataatgatcgaggaggtgatgagatccagatggagtagaagaatgctgatgactggaacactggctgtgttcttccttctcataatgggacaattgacatggaacgatctgatcagattatgcatcatggttggagccaacgcttccgacaggatggggatgggaacgacgtacctagccctgatggccacttttaaaatgagaccgatgttcgctgtagggctattatttcgcagactaacatccagagaagttcttcttctaacaattggattgagtctagtggcatctgtggagttaccaaattccttggaggagctgggggatggacttgcaatgggcattatgattttaaaattattgactgactttcaatcacatcagctgtgggctaccttgctgtccttgacatttatcaaaacaacgttttccttgcactacgcatggaagacaatggctatggtactgtcaattgtatctctcttccctttatgcctgtccacgacctcccaaaaaacaacatggcttccggtgctattgggatcccttggatgcaaaccactaaccatgtttcttatagcagaaaacaaaatctggggaaggagaagttggcccctcaatgaaggaatcatggctgttggaatagtcagcatcctactaagttcactcctcaaaaatgatgtaccgctagctgggccactaatagctggaggcatgctaatagcatgttatgttatatctggaagctcagccgacctatcattagagaaagcggctgaggtctcctgggaagaagaagcagaacactctggtgcctcacacaacatattagtggaagtccaagatgatggaaccatgaagataaaggatgaagagagagatgacacgctaaccattctccttaaagcaactctgttagcagtttcaggggtgtacccattatcaataccagcgacccttttcgtgtggtacttttggcagaaaaagaaacagagatctggagtgttatgggacacacccagccctccagaagtggaaagagcagttcttgatgatggtatctatagaattatgcagagaggactgttgggcaggtcccaagtaggggtaggagttttccaagaaaacgtgttccacacaatgtggcatgtcaccaggggagctgtactcatgtatcaagggaagagattggaaccgagctgggccagtgtcaaaaaagacctgatctcatatggaggaggttggaggcttcaaggatcctggaacacaggagaagaagtgcaggtgattgctgttgaaccagggaaaaaccccaaaaatgtacaaacagcgccgggcacctttaagacccctgaaggtgaagttggagccattgccctagactttaaacctggcacatctggatctcccatcgtgaacagagaaggaaaaatagtaggtctttatggaaatggagtagtgacaacaagtggaacctacgtcagtgccatagctcaagccaaagcatcacaagaagggcccctaccagagattgaagacgaggtgtttaggaaaagaaacttaacaataatggacctacatccaggatcggggaaaacaagaagatatcttccagccatagtccgtgaggccataaaaaggaagctgcgcacactaatcctggctcccacaagggttgtcgcttccgaaatggcagaggcgctcaagggaatgccaataaggtaccaaacaacagcagtgaagagtgaacatacaggaaaagagatagttgacctcatgtgtcacgccactttcaccatgcgcctcctgtctcccgtaagagttcccaattacaacatgatcatcatggatgaagcacatttcaccgatccatccagtatagcggccagagggtacatctcaacccgagtgggcatgggtgaagcagctgcaatcttcatgacagccactcccccaggatcagtggaggcctttccacagagcaacgcagttatccaagatgaggaaagagacattcctgagagatcatggaactcaggctatgagtggatcactgacttcccaggtaaaacagtttggtttgttccaagcattaaatcaggaaatgacattgccaactgcttaagaaagaatgggaaacgggtgattcaattgagcaggaaaacctttgatacagagtaccaaaaaacaaaaaacaacgactgggactacgtcgtcacaacagacatctccgaaatgggagcaaatttccgagccgacagggtgatagacccaagacggtgtctgaaaccggtaatactaaaagatggtccagagcgtgtcattttagcaggaccaatgccagtgactgtggccagtgccgctcagaggagaggaagaattggaaggaaccacaataaggaaggtgatcagtacatctacatgggacagcctttaaacaacgatgaagatcacgctcactggacagaagcaaaaatgctccttgataatataaacacaccagaagggattatcccagccctctttgagccagagagagaaaagagtgcagcaatagacggggaatacagactgcggggtgaagcaaggaaaacgtttgtggagctcatgagaagaggagatctacctgtctggctatcctacaaagttgcctcagaaggcttccagtactctgacagaagatggtgctttgacggggaaaggaacaaccaggtgttggaggagaacatggacgtggagatctggacaaaagaaggagaaagaaagaaactacgaccccgctggctggatgccagaacatactcagacccactagccctgcgcgagtttaaagagtttgcagcagggagaagaagcgtctcaggtgatttaatattagaaatagggaagcttccacaacacttgacgcaaagggcccagaatgccctggacaacctggttatgttgcacaactccgaacaaggaggcagagcctatagacatgcaatggaagaactgccagacaccatagaaacgttgatgctcctagctttgatagctgtgttaactggtggagtgacactgttcttcctatcaggaaggggcctagggaaaacatctatcggcctactctgcgtaatggcttcaagcgtactgctatggatggccagtgtggagccccattggatagcggcctccatcatactggagttcttcctgatggtgctgcttattccagagccagacagacaacgcactccgcaggacaaccagctggcatatgtggtgataggtttgttattcatgatactgacagtagcagccaatgagatgggactgctggaaaccacaaagaaagacttagggattggccatgtggctgttgaaaatcaccaccatgccgcaatgctggacgtagacttacatccagcttcagcctggaccctctatgcagtggccacaacaattatcactcccatgatgaggcacacaatcgaaaacacaacggcaaacatttccctgacagccattgcaaaccaggcagctatattgatgggacttgacaaaggatggccaatatcgaagatggacataggagttccacttctcgccttggggtgctattcccaggtgaatccactgacgctgacagcggcggtattgatgctagtggctcattacgccataattggacctggactgcaagcaaaagctactagagaagctcaaaaaaggacagcggccggaataatgaaaaatccaaccgttgatggaattgttgcaatagatttggaccctgtggtttatgatgcaaaatttgaaaaacaactaggccaaataatgttgttgatactatgcacatcacagatcctcttgatgcggactacatgggccttgtgcgagtccatcacactggccactggacctctgaccacgctttgggagggatctccaggaaaattttggaacaccacgatagcggtttccatggcaaacattttcagaggaagttatctagcaggagcaggtctggccttctcattaatgaaatctctaggaggaggtaggagaggcacgggagcccaaggggaaacactgggagagaaatggaaaagacagctgaaccaactgagcaagtcagaatttaacacctataaaaggagtgggattatggaagtggacagatccgaagccaaagagggattgaaaagaggagaaacaaccaaacatgcagtgtcgagaggaaccgctaaactgaggtggttcgtggagaggaaccttgtgaaaccagaagggaaagtcatagacctcggttgtggaagaggtggctggtcatactattgcgctgggctgaagaaagtcacagaagtgaaggggtatacaaaaggaggacctggacatgaggaaccaatcccaatggcgacctatggatggaacctagtaaagctgcactctgggaaagacgtattttttataccacctgagaaatgtgacacccttttgtgtgatattggtgagtcctctccaaacccaactatagaggaaggaagaacgctacgcgtcctaaagatggtggaaccatggctcagaggaaaccaattttgcataaaaattctgaatccctacatgccaagtgtggtggaaactctggagcaaatgcaaagaaaacatggaggaatgctagtgcgaaatccactttcaagaaattctactcatgaaatgtattgggtttcatgtggaacaggaaacattgtgtcagcagtaaacatgacatctagaatgttgctaaatcgattcacaatggctcacaggaaaccaacatatgaaagagacgtggacctaggcgccggaacaagacatgtggcagtggaaccagaggtagccaacctagatatcattggccagaggatagagaacataaaacatgaacataagtcaacatggcattatgatgaggacaatccatataaaacatgggcctatcatggatcatatgaggtcaagccatcaggatcagcctcatccatggtcaatggcgtggtgaaactgctcaccaaaccatgggatgtcatccctatggtcacacaaatagccatgactgacactacaccctttggacaacagagggtgtttaaagagaaagttgacacacgcacaccaaaagcaaaacggggcacagcacaaatcatggaggtgacagccaagtggttatggggttttctttctagaaacaagaaaccaagaatttgcacaagagaggagttcacaagaaaagttaggtcaaacgcagccattggagcagtgttcgttgatgaaaatcaatggaactcagcaaaagaagcagtggaagatgagcggttctgggaccttgtgcatagagagagggagcttcacaaacagggaaaatgtgctacgtgtgtttacaacatgatggggaagagagagaaaaagctaggagagttcggaaaggcaaaaggaagtcgtgcaatatggtacatgtggttgggagcacgctttctagagttcgaagctcttggtttcatgaacgaagatcactggttcagcagagagaattcactcagcggagtggaaggagaaggactccacaaacttggatatatactcagagacatatcaaagattccagggggaaacatgtatgcagatgacacagccggatgggatacaaggataacagaggatgaccttcagaatgaggccagaattactgacatcatggaacccgaacatgccctcctggctaagtcaatcttcaagttaacctaccaaaataaggtggtaagggtacagagaccagcaaaaaatggaaccgtgatggatgtcatatccagacgtgaccagagaggaagtggtcaggtcggaacttatggcttaaacactttcaccaacatggaagcccagctgataagacaaatggagtctgagggaatcttttcacccagcgaattagagaccccaaatttagccgagagagttctcgactggctggaaaaatatggcgtcgaaaggctgaaaagaatggcaatcagcggagatgactgcgtagtgaaaccaattgatgataggtttgcaacagccttgacagctctgaatgatatgggaaaagtaagaaaagatataccacaatgggaaccttcaaaaggatggaatgattggcaacaagtgcctttttgttcacaccacttccaccagctgattatgaaggatgggagggaaatagtggtgccatgccgcaaccaagatgaacttgtgggtagggctagagtatcacaaggtgctggatggagcctgagagaaactgcatgcctaggcaagtcatatgcacaaatgtggcagctgatgtacttccacaggagagacctgagactagccgctaatgctatctgttcagccgttccagttgattggatcccaaccagccgtaccacctggtcgatccatgcccatcaccaatggatgacaacagaagacatgctgtcagtgtggaatagggtttggatagaggaaaacccatggatggaggacaaaacccacatatccagttggggagatgttccatatttaggaaaaagggaagaccaatggtgtggatccctgataggcttaacagcaagggccacctgggccaccaacatacaagtggccataaaccaagtgagaagactaattgggaatgagaattatctagattacatgacatcaatgaagagattcaagaacgagagtgatcccgaaggggcactctggtgagtcaacacatttacaaaataaaggaaaataagaaatcaaacaaggcaagaagtcaggccggattaagccatagtacggtaagagctatgctgcctgtgagccccgtctaaggacgtaaaatgaagtcaggccgaaagccacggcttgagcaaaccgtgctgcctgtagctccatcgtggggatgtaaaaacctgggaggctgcaacccatggaagctgtacgcatggggtagcagactagtggttagaggagacccctcccgaaacataacgcagcagcggggcccaacaccaggggaagctgtaccctggtggtaaggactagaggttagaggagaccccccgcataacaataaacagcatattgacgctgggagagaccagagatcctgctgtctctacagcatcattccaggcacagaacgccagaaaatggaatggtgctgttgaatcaacaggttct

SEQ ID NO: 3 - DNA, 10725 bp, Dengue virus
  source 1..10725: mol_type = genomic DNA
agttgttagtctacgtggaccgacaaagacagattctttgagggagctaagctcaacgtagttctaacagttttttaattagagagcagatctctgatgaataaccaacgaaaaaaggcgagaagtacgcctttcaatatgctgaaacgcgagagaaaccgcgtgtcaactgtgcaacagctgacaaagagattctcacttggaatgctgcaaggacgcggaccattaaaactgttcatggcccttgtggcgttccttcgtttcctaacaatcccaccaacagcagggatactaaaaagatggggaacgatcaaaaaatcaaaagctatcaatgttttgagagggttcaggaaagagattggaaggatgctgaacatcttgaacaagagacgcaggacagcaggcgtgattgttatgttgattccaacagcgatggcgttccatttaaccacacgcaatggagaaccacacatgatcgttggtaggcaggagaaagggaaaagtcttctgttcaaaacagaggatggtgttaacatgtgtactctcatggccatagaccttggtgaattgtgtgaagatacaatcacgtacaagtgtcctctcctcagacaaaatgaaccagaagacatagattgttggtgcaactctacgtccacatgggtaacttatgggacatgtaccaccacaggagaacacagaagagaaaaaagatcagtggcgctcgttccacatgtaggtatgggactggagacacgaactgaaacatggatgtcatcagaaggggcctggaaacatgttcagagaattgaaacctggatcttgagacatccaggttttaccataatggcagcaatcctggcatacaccataggaacgacacatttccaaagggccttgattttcattttactgacagctgtcgctccttcaatgacaatgcgctgcataggaatatcaaatagagacttcgtagaaggggtttcaggaggaagctgggttgacatagtcttagaacatggaagttgtgtgacgacgatggcaaaaaacaaaccaacattggattttgaactgataaaaacagaagccaaacaacctgccactctaaggaagtactgtatagaagcaaagctgaccaacacaacaacagaatcgcgttgcccaacacaaggggaacccagtctaaatgaggagcaggacaaaaggttcatctgcaaacactccatggtagacagaggatggggaaatggatgtggattatttggaaagggaggcattgtgacctgtgctatgtttacatgcaaaaagaacatggaaggaaaagtcgtgcagccagaaaatttggaatacaccatcgtgataacacctcactcaggagaggagcacgctgtaggtaatgacacaggaaagcatggcaaggaaatcaaaataacaccacagagctccatcacagaagcagaactgacaggctatggcactgtcacgatggagtgctctccgagaacgggcctcgacttcaatgagatggtactgctgcagatggaagacaaagcttggctggtgcacaggcaatggttcctagacctgccgttaccatggctacccggagcggacacacaaggatcaaattggatacagaaagagacattggtcactttcaaaaatccccacgcgaagaaacaggatgtcgttgtcttagggtctcaagaaggggccatgcacacggcactcacaggggccacagaaatccagatgtcatcaggaaacttactgttcacaggacatctcaagtgcaggctgagaatggacaaactacagctcaaaggaatgtcatactctatgtgtacaggaaagtttaaaattgtgaaggaaatagcagaaacacaacatggaacaatagttatcagagtacaatatgaaggggacggttctccatgcaagatcccttttgagataacagatttggaaaaaagacacgtcttaggtcgcttgattacagttaacccaatcgtaacagaaaaagatagcccagtcaacatagaagcagaacctccattcggagacagctacatcattataggagtagagccgggacaattgaaactcaattggtttaagaagggaagttccatcggccaaatgtttgagacaacaatgagaggagcaaagagaatggccattttaggtgacacagcctgggactttggatccctgggaggagtgtttacatctataggaaaggctctccaccaagttttcggagcaatctatggggctgcttttagtggggtctcatggactatgaaaatcctcataggagtcatcatcacatggataggaatgaattcacgtagcacctcactgtctgtgtcgctagtattggtgggcgttgtgacactgtacctgggagctatggtgcaagctgatagtggttgcgttgtgagctggaaaaataaagaactgaaatgtggcagcgggatcttcatcacagataacgtacacacatggacagaacaatataagttccaaccagaatccccttcaaaactagcttcagctatccaaaaagctcatgaagagggcatttgtggaatccgctcagtaacaagattggagaatctgatgtggaaacaaataacaccagaattgaatcatattctatcagaaaatgaggtaaagttgaccattatgacaggagacattagaggaatcatgcaggcaggaaaacgatccttgcggccccagcccactgagctgaagtactcatggaaaacatggggaaaggcgaaaatgctctccacagagtctcacaatcagacctttcttattgatggccctgaaacagcagaatgccccaacacaaacagagcctggaactcgctggaagttgaagactatggttttggagttttcaccaccaatatatggctgaaattgagagaaaaacaggatgtattttgtgactcaaaactcatgtcagcggccattaaagacaacagagccgttcatgctgatatgggttattggatagaaagtgcactcaatgacacatggaagatggagaaagcctccttcattgaagttaaaagctgccactggccaaagtcacacaccctttggagcaatggagtattagaaagtgagatgataatcccaaaaaattttgccgggccagtgtcacaacacaactacagaccaggctaccatacacaaacagcaggaccttggcatctaggtaagcttgagatggactttgatctctgcgaaggaactacagtggtggtgactgaggactgtggaaatagaggaccctctttaagaacgaccactgcctctggaaaactcataacagaatggtgctgccgatcctgcacactaccacctctaagatacagaggtgaggatggatgctggtacgggatggaaatcagaccattgaaagagaaagaagagaatttggtcaactccttggtcacagccggacatgggcagattgacaacttttcactaggagtcttgggaatggcactgttcctggaagaaatgctcaggacccgaataggaacgaaacatgcaatactgctagttgcagtatcttttgtgacattgattactgggaacatgtcttttagagacctgggaagagtgatggttatggtgggcgctaccatgacggatgacataggtatgggagtgacttatcttgccctactagcagcttttaaggttagaccaacttttgcagctggactactcttaagaaaactgacctccaaggaattgatgatggccaccataggaatcgcactcctttcccaaagcaccataccagagaccattcttgaactgactgatgcattagccctgggcatgatggtcctcaaaatagtgagaaatatggaaaaataccaattggcagtgactatcatggctatttcatgtgtcccaaatgcagtgatactgcaaaacgcatggaaggtgagttgcacaatattggcagcggtgtccgtttcaccactgctcttaacatcctcacagcagaaagcggattggataccactggcattgacgataaaaggtctcaatccaacagccatttttttaacaactctctcgaggaccagcaagaaaaggagctggccgctaaatgaagctatcatggcagttgggatggtgagcattttagccagttctctcctaaagaatgatattcctatgacaggtccattagtggctggaggactcctcaccgtatgttacgtgctcactggacgatcggccgatttggaactggagagagctgccgatgtaaaatgggaagatcaggcagaaatatcaggaagcagcccaatcctgtcaataacaatatcagaagatggcagcatgtcgataaaaaatgaagaggaagaacaaacactgaccatactcatcagaacgggattgttggtgatctcaggagtctttccagtatcgataccaattacggcagcagcatggtacctgtgggaagtaaagaaacaacgggctggagtactgtgggacgtcccttcacccccaccagtggaaaaagccgaactggaggatggagcctacagaatcaagcaaagagggatccttggatattctcagattggagccggagtttacaaagaaggaacattccatacaatgtggcacgtcacacgtggtgctgttctgatgcatagagggaagaggattgaaccatcatgggcagatgtcaagaaagacctaatatcatatggaggaggctggaagctagaaggagaatggaaggaaggagaggaagtccaagtcctggcattggaacctggaaaaaatccaagagccgtccaaacgaaacctggaatattcaaaaccaacaccggaaccataggcgccgtatctctggacttttcccctggaacgtcaggatctccaatcgtcgacagaaaaggaaaagttgtgggtctttacggtaatggtgttgtcacaaggagtggagcatatgtaagtgctatagcccagaccgaaaaaagcattgaagacaatccagagatcgaagatgacattttccgaaagaaaagattgaccatcatggacctccatccaggagcaggaaagacaaaaagataccttccagccatagttagagaagccataaaacgtggcttgagaacattgatcctggctcccactagagtagtggcagctgaaatggaggaagctcttagaggacttccaataagataccaaactacagccatcaaaaccgagcataccgggcgggagatcgtggacctaatgtgtcatgccacatttactatgaggctgttatcaccagtcagagtgccaaattacaacctgatcatcatggacgaagcccacttcacagacccagcaagtatagcagctagaggatacatttcaactcgagtagagatgggtgaagcagccgggattttcatgacagccactcctccgggaagtagagacccatttcctcagagcaatgcaccaattatggatgaggaaagagaaatccctgagcgttcatggaattcaggacacgaatgggtcacggattttaaggggaagactgtttggtttgttccaagtataaaagcaggaaatgatatagcagcttgtcttaggaaaaatggaaagaaagtgatacaactcagtaggaagacttttgactctgagtatgttaagactagagccaatgattgggactttgtggtcacaactgacatttcagaaatgggtgccaacttcaaggctgagagggttatagaccccagacgttgcatgaaaccagttatactaacagatggcgaggagcgggtgatcttggctggacctatgccagtgacccactctagtgcagcgcaaagaagagggagaataggaagaaatccaaaaaatgaaaatgaccagtacatatacatgggggaacctcttgaaaatgatgaagactgtgcacattggaaagaagctaaaatgctcctagataacatcaacacacctgaaggaatcattcctagtatgttcgaaccagagcgtgaaaaagtggatgccattgatggtgaataccgtttgagaggagaagcaaggaaaacctttgtggacctaatgagaagaggggacttaccagtctggttggcctacaaagtggcagctgaaggcatcaactacgcagacagaaagtggtgttttgatggaattaagaacaaccaaatactggaagaaaatatggaagtggaaatctggacaaaagaaggggaaaggaaaaaattaaaacccagatggttggatgctaggatctattctgacccactagcactaaaagaattcaaggaatttgcagctggaagaaaatctttgaccctgaacctaatcacagaaatgggtaggcttccaactttcatgactcagaaagcaagaaacgcactggacaacctggctgtgctgcatacggctgaggcaggtggaagggcgtacaatcatgctctcagtgaactgccggagaccctggagacactgctcctactgacacttctggcaacagtcacaggaggaatcttcttattcttaatgagcggaaaaggtatagggaagatgaccctgggaatgtgttgcataatcacggctagtatcctcctatggtatgcacagatacaaccacactggatagcagcttcaataatactggagttttttctcatagttttgctcattccagaaccagaaaaacagagaacaccccaagacaaccaattgacctacgttgtcatagccatcctcacagtggtggccgcaaccatggcaaacgagatgggtttcctggaaaaaaccaagaaagacctcggattgggaagcattacaacccaggaatctgagagcaatatcctggacatagatctacgccctgcatcagcatggacgctgtatgccgtagctacaacatttgtcacaccaatgttgagacatagcattgaaaattcctcagtgaatgtctccctaacagccattgctaaccaagctacagtgctaatgggtcttgggaaaggatggccattgtcaaagatggacattggagttcccctccttgccattggatgctattcacaagtcaaccctataactctcacagcagctctccttttattggtagcacattatgccattatagggccaggacttcaagcaaaagcaaccagagaagcccagaaaagagcagcagcaggcatcatgaaaaacccaacagtcgatggaataacagtgattgacctagaaccaataccctatgatccaaaatttgaaaagcagttaggacaagtaatgctcctaatcctctgcgtgactcaagtattaatgatgaggactacatgggctttatgtgaggctctaaccctagcgaccgggcccatctccacactgtgggaaggaaatccagggaggttttggaacactaccattgcagtgtcaatggctaacatctttagggggagctacttggccggagctggacttctcttttccatcatgaaaaacacaacaaacacaagaagaggaactggcaacataggagagacacttggagaaaaatggaaaagtcgattaaacgcactggggaaaagtgaatttcaaatctacaagaaaagtggaatccaggaagtggatagaaccctagcaaaagaaggtatcaaaagaggagaaacggaccaccatgctgtgtcgcgaggttcagcaaaactgagatggttcgtcgagagaaatatggtcacaccggaagggaaggtggtggatctcggttgcggcagagggggctggtcatactattgcgggggactaaagaatgtaagagaagtcaaaggcctaacaaaaggaggaccaggacatgaagaacccatccccatgtcaacatatgggtggaatctagtgcgtctgcaaagtggagttgacgttttcttcaccccgccagaaaagtgtgatacattgttgtgtgacataggggagtcgtcaccaaatcccacgatagaagcaggacgaacactcagagtcctcaacttagtggaaaattggttgaacaataacacccaattttgcataaaggtcctcaacccatatatgccttcagtcatagaaaaaatggaagcattacaaaggaaatatggaggagccttagtgaggaatccactctcacgaaactccacgcatgaaatgtactgggtatctaatgccaccgggaacatagtgtcatcagtgaacatgatttcaaggatgttgattaacagattcacaatgaaacacaagaaagccacttacgagccagatgttgacctaggaagtggaacccgcaacattggaattgaaagtgagataccaaatctagacataataggaaagagaatagagaaaataaaacaagagcatgaaacatcatggcactatgatcaagaccacccatacaaaacgtgggcttaccatggcagctatgaaacaaaacaaactggatcagcatcatctatggtgaacggagtggtcagattgctgacaaaaccttgggacgtcgtccctatggtgacacagatggcaatgacagacacgactccttttggacaacagcgcgttttcaaagagaaagtagacacgagaacccaagaaccgaaggaaggcacaaagaaactgatgaaaattacggcagagtggctttggaaagaactaggaaagaaaaagacacctaggatgtgtaccagagaagaattcacaagaaaagtgagaagcaatgcagccttgggggccatattcactgatgagaacaaatggaaatcggcacgtgaggctgttgaagatggtaggttctgggagctggttgacagggaaagaaatctccatcttgaaggaaagtgtgaaacatgtgtgtacaacatgatgggaaaaagagagaagaaactaggggagttcggcaaggcaaaaggtagcagagccatatggtacatgtggcttggagcacgcttcttagagtttgaagccctaggattcctgaatgaagatcactggttctccagagggaactccctgagtggagtggaaggagaagggctgcacaggctaggctacattttaagagacgtgggcaagaaggaagggggggcaatgtacgccgatgatacagcaggatgggacacaagaatcacactagaagacttaaaaaatgaagaaatggtaacgaaccacatgaaaggagaacacaagaaactagccgaggccatattcaaactaacgtaccaaaacaaggtggtgcgtgtgcaaagaccaacaccaagaggtacagtaatggatatcatatcgagaagagaccaaagaggcagtgggcaagtcggcacctatggccttaataccttcaccaatatggaagcccaattaattagacagatggagggagaaggaatcttcaaaagcattcagcacctgacagccacagaagaaatcgctgtacagaactggctagcaagagtggggcgtgaaaggctatcaagaatggcaatcagtggagatgattgtgttgtaaaacctatagatgacagatttgcaagtgctttaacagctctaaatgacatgggaaaagttagaaaagatatacaacaatgggaaccttcaagaggatggaacgattggacacaagtgcctttctgttcacaccactttcatgagttagtcatgaaagatggtcgcgtgctcgtagtcccatgcagaaaccaagatgaactgattggtagagcccgaatttcccagggagctgggtggtctttgaaagagacggcctgtttgggaaagtcttacgcccaaatgtggactctgatgtacttccacagacgtgacctcagactggcggcaaatgccatctgctcggcagtcccgtcacattgggttccaacaagtcgaacaacctggtccatacacgctaagcatgaatggatgacgacggaagacatgctggcagtctggaacagggtgtggatccaagaaaacccgtggatggaagataaaactccagtggaatcatgggaagaagtcccatacttgggaaaaagagaagaccaatggtgcggctcattgattgggctaacaagcagggctacctgggcaaagaacatccaaacagcaataaatcaagtcagatcccttataggcaatgaggaatacacagactacatgccatccatgaagagatttagaagggaagaggaagaggcaggtgtcctgtggtagaaggcaaaactaacatgaaacaaggctaaaagtcaggtcggattaagccatagtacggaaaaaactatgctacctgtgagccccgtccaaggacgttaaaagaagtcaggccatcacaaaatgccacagcttgagtaaactgtgcagcctgtagctccacctgaggaggtgtaaaaaacctgggaggccacaaaccatggaagctgtacgcatggcgtagtggactagcggttagaggagacccctcccttacaaatcgcagcaaacaacgggggcccaaggtgagatgaagctgtaatctcactggaaggactagaggttagaggagacccccccaaaacaaaaaacagcatattgacgctgggaaagaccagagatcctgctgtctcctcagcatcattccaggcacagaacgccagaaaatggaatggtgctgttgaatcaacaggttct

SEQ ID NO: 4 - DNA, 10725 bp, Dengue virus
  source 1..10725: mol_type = genomic DNA
agttgttagtctacgtggaccgacaaagacagattctttgagggagctaagctcaacgtagttctaacagttttttaattagagagcagatctctgatgaataaccaacgaaaaaaggcgagaagtacgcctttcaatatgctgaaacgcgagagaaaccgcgtgtcaactgtgcaacagctgacaaagagattctcacttggaatgctgcaaggacgcggaccattaaaactgttcatggcccttgtggcgttccttcgtttcctaacaatcccaccaacagcagggatactaaaaagatggggaacgatcaaaaaatcaaaagctatcaatgttttgagagggttcaggaaagagattggaaggatgctgaacatcttgaacaagagacgcaggacagcaggcgtgattgttatgttgattccaacagcgatggcgttccatttaaccacacgcaatggagaaccacacatgatcgttggtaggcaggagaaagggaaaagtcttctgttcaaaacagaggatggtgttaacatgtgtactctcatggccatagaccttggtgaattgtgtgaagatacaatcacgtacaagtgtcctctcctcagacaaaatgaaccagaagacatagattgttggtgcaactctacgtccacatgggtaacttatgggacatgtaccaccacaggagaacacagaagagaaaaaagatcagtggcgctcgttccacatgtaggtatgggactggagacacgaactgaaacatggatgtcatcagaaggggcctggaaacatgttcagagaattgaaacctggatcttgagacatccaggttttaccataatggcagcaatcctggcatacaccataggaacgacacatttccaaagggccttgattttcattttactgacagctgtcgctccttcaatgacaatgagatgcatagggatatcgaatcgcgatttcgtcgaaggcgtatccggagggtcatgggtcgacatcgtactcgaacacggatcatgcgttacgactatggctaagaataagcctacactagacttcgaactgattaagacagaggctaagcaaccggcaacattgcgtaagtactgtatcgaagcgaaactgactaacactacaaccgaatctagatgccctacacagggcgaacctagtctgaacgaagagcaagacaaaaggtttatatgcaaacactctatggtcgatcgcggatggggaaacggatgcggattgttcggtaaggggggaatcgttacatgcgctatgtttacatgtaaaaaaaatatggagggaaaggtcgtgcaaccagagaatctcgaatatacaatcgtaatcacaccgcatagcggagaggaacacgcagtcggaaacgataccggaaaacacggaaaagagattaagattacaccacagagctccataaccgaagccgaactgacagggtacggaacagtgacaatggaatgctcacctagaacaggcctagactttaacgaaatggtgttactgcaaatggaagacaaagcatggttagtgcataggcaatggtttttagacctaccactaccatggttgcccggagccgatacacagggatcgaactggatacagaaagagacactcgttacgtttaaaaacccacacgctaaaaaacaggacgtagtcgtactcggatcacaggaaggcgcaatgcataccgcattgacaggcgctacagagatacagatgtctagcggaaatctgttgtttacagggcatctgaaatgtagactgagaatggacaaactgcaattgaagggaatgtcatactctatgtgtacgggtaagtttaagatagtcaaagagatagccgaaacacaacacggaacaatcgtaattagggtgcaatacgaaggcgacgggtcaccatgtaagataccattcgaaattacagacctcgaaaaaagacacgtactcggaagactgataacagtgaatccgatcgttacggaaaaagactcacccgttaatatcgaagccgaaccaccattcggagactcatacataataatcggagtcgaacccggacaattgaaactgaattggtttaaaaaagggtcatcaatcggacaaatgttcgaaacaactatgagaggcgctaagcgtatggctatactcggagacacagcatgggacttcggatccttagggggagtgtttacgtcaatcggtaaggcactacaccaggtattcggagcgatatacggagccgcatttagcggagtgtcgtggacaatgaagatactgatcggagtgataatcacatggatcggaatgaatagtaggtctacaagtctatccgttagcttagtgttagtcggagtcgttacactgtatctaggcgctatggtgcaagccgatagtggttgcgttgtgagctggaaaaataaagaactgaaatgtggcagcgggatcttcatcacagataacgtacacacatggacagaacaatataagttccaaccagaatccccttcaaaactagcttcagctatccaaaaagctcatgaagagggcatttgtggaatccgctcagtaacaagattggagaatctgatgtggaaacaaataacaccagaattgaatcatattctatcagaaaatgaggtaaagttgaccattatgacaggagacattagaggaatcatgcaggcaggaaaacgatccttgcggccccagcccactgagctgaagtactcatggaaaacatggggaaaggcgaaaatgctctccacagagtctcacaatcagacctttcttattgatggccctgaaacagcagaatgccccaacacaaacagagcctggaactcgctggaagttgaagactatggttttggagttttcaccaccaatatatggctgaaattgagagaaaaacaggatgtattttgtgactcaaaactcatgtcagcggccattaaagacaacagagccgttcatgctgatatgggttattggatagaaagtgcactcaatgacacatggaagatggagaaagcctccttcattgaagttaaaagctgccactggccaaagtcacacaccctttggagcaatggagtattagaaagtgagatgataatcccaaaaaattttgccgggccagtgtcacaacacaactacagaccaggctaccatacacaaacagcaggaccttggcatctaggtaagcttgagatggactttgatctctgcgaaggaactacagtggtggtgactgaggactgtggaaatagaggaccctctttaagaacgaccactgcctctggaaaactcataacagaatggtgctgccgatcctgcacactaccacctctaagatacagaggtgaggatggatgctggtacgggatggaaatcagaccattgaaagagaaagaagagaatttggtcaactccttggtcacagccggacatgggcagattgacaacttttcactaggagtcttgggaatggcactgttcctggaagaaatgctcaggacccgaataggaacgaaacatgcaatactgctagttgcagtatcttttgtgacattgattactgggaacatgtcttttagagacctgggaagagtgatggttatggtgggcgctaccatgacggatgacataggtatgggagtgacttatcttgccctactagcagcttttaaggttagaccaacttttgcagctggactactcttaagaaaactgacctccaaggaattgatgatggccaccataggaatcgcactcctttcccaaagcaccataccagagaccattcttgaactgactgatgcattagccctgggcatgatggtcctcaaaatagtgagaaatatggaaaaataccaattggcagtgactatcatggctatttcatgtgtcccaaatgcagtgatactgcaaaacgcatggaaggtgagttgcacaatattggcagcggtgtccgtttcaccactgctcttaacatcctcacagcagaaagcggattggataccactggcattgacgataaaaggtctcaatccaacagccatttttttaacaactctctcgaggaccagcaagaaaaggagctggccgctaaatgaagctatcatggcagttgggatggtgagcattttagccagttctctcctaaagaatgatattcctatgacaggtccattagtggctggaggactcctcaccgtatgttacgtgctcactggacgatcggccgatttggaactggagagagctgccgatgtaaaatgggaagatcaggcagaaatatcaggaagcagcccaatcctgtcaataacaatatcagaagatggcagcatgtcgataaaaaatgaagaggaagaacaaacactgaccatactcatcagaacgggattgttggtgatctcaggagtctttccagtatcgataccaattacggcagcagcatggtacctgtgggaagtaaagaaacaacgggctggagtactgtgggacgtcccttcacccccaccagtggaaaaagccgaactggaggatggagcctacagaatcaagcaaagagggatccttggatattctcagattggagccggagtttacaaagaaggaacattccatacaatgtggcacgtcacacgtggtgctgttctgatgcatagagggaagaggattgaaccatcatgggcagatgtcaagaaagacctaatatcatatggaggaggctggaagctagaaggagaatggaaggaaggagaggaagtccaagtcctggcattggaacctggaaaaaatccaagagccgtccaaacgaaacctggaatattcaaaaccaacaccggaaccataggcgccgtatctctggacttttcccctggaacgtcaggatctccaatcgtcgacagaaaaggaaaagttgtgggtctttacggtaatggtgttgtcacaaggagtggagcatatgtaagtgctatagcccagaccgaaaaaagcattgaagacaatccagagatcgaagatgacattttccgaaagaaaagattgaccatcatggacctccatccaggagcaggaaagacaaaaagataccttccagccatagttagagaagccataaaacgtggcttgagaacattgatcctggctcccactagagtagtggcagctgaaatggaggaagctcttagaggacttccaataagataccaaactacagccatcaaaaccgagcataccgggcgggagatcgtggacctaatgtgtcatgccacatttactatgaggctgttatcaccagtcagagtgccaaattacaacctgatcatcatggacgaagcccacttcacagacccagcaagtatagcagctagaggatacatttcaactcgagtagagatgggtgaagcagccgggattttcatgacagccactcctccgggaagtagagacccatttcctcagagcaatgcaccaattatggatgaggaaagagaaatccctgagcgttcatggaattcaggacacgaatgggtcacggattttaaggggaagactgtttggtttgttccaagtataaaagcaggaaatgatatagcagcttgtcttaggaaaaatggaaagaaagtgatacaactcagtaggaagacttttgactctgagtatgttaagactagagccaatgattgggactttgtggtcacaactgacatttcagaaatgggtgccaacttcaaggctgagagggttatagaccccagacgttgcatgaaaccagttatactaacagatggcgaggagcgggtgatcttggctggacctatgccagtgacccactctagtgcagcgcaaagaagagggagaataggaagaaatccaaaaaatgaaaatgaccagtacatatacatgggggaacctcttgaaaatgatgaagactgtgcacattggaaagaagctaaaatgctcctagataacatcaacacacctgaaggaatcattcctagtatgttcgaaccagagcgtgaaaaagtggatgccattgatggtgaataccgtttgagaggagaagcaaggaaaacctttgtggacctaatgagaagaggggacttaccagtctggttggcctacaaagtggcagctgaaggcatcaactacgcagacagaaagtggtgttttgatggaattaagaacaaccaaatactggaagaaaatatggaagtggaaatctggacaaaagaaggggaaaggaaaaaattaaaacccagatggttggatgctaggatctattctgacccactagcactaaaagaattcaaggaatttgcagctggaagaaaatctttgaccctgaacctaatcacagaaatgggtaggcttccaactttcatgactcagaaagcaagaaacgcactggacaacctggctgtgctgcatacggctgaggcaggtggaagggcgtacaatcatgctctcagtgaactgccggagaccctggagacactgctcctactgacacttctggcaacagtcacaggaggaatcttcttattcttaatgagcggaaaaggtatagggaagatgaccctgggaatgtgttgcataatcacggctagtatcctcctatggtatgcacagatacaaccacactggatagcagcttcaataatactggagttttttctcatagttttgctcattccagaaccagaaaaacagagaacaccccaagacaaccaattgacctacgttgtcatagccatcctcacagtggtggccgcaaccatggcaaacgagatgggtttcctggaaaaaaccaagaaagacctcggattgggaagcattacaacccaggaatctgagagcaatatcctggacatagatctacgccctgcatcagcatggacgctgtatgccgtagctacaacatttgtcacaccaatgttgagacatagcattgaaaattcctcagtgaatgtctccctaacagccattgctaaccaagctacagtgctaatgggtcttgggaaaggatggccattgtcaaagatggacattggagttcccctccttgccattggatgctattcacaagtcaaccctataactctcacagcagctctccttttattggtagcacattatgccattatagggccaggacttcaagcaaaagcaaccagagaagcccagaaaagagcagcagcaggcatcatgaaaaacccaacagtcgatggaataacagtgattgacctagaaccaataccctatgatccaaaatttgaaaagcagttaggacaagtaatgctcctaatcctctgcgtgactcaagtattaatgatgaggactacatgggctttatgtgaggctctaaccctagcgaccgggcccatctccacactgtgggaaggaaatccagggaggttttggaacactaccattgcagtgtcaatggctaacatctttagggggagctacttggccggagctggacttctcttttccatcatgaaaaacacaacaaacacaagaagaggaactggcaacataggagagacacttggagaaaaatggaaaagtcgattaaacgcactggggaaaagtgaatttcaaatctacaagaaaagtggaatccaggaagtggatagaaccctagcaaaagaaggtatcaaaagaggagaaacggaccaccatgctgtgtcgcgaggttcagcaaaactgagatggttcgtcgagagaaatatggtcacaccggaagggaaggtggtggatctcggttgcggcagagggggctggtcatactattgcgggggactaaagaatgtaagagaagtcaaaggcctaacaaaaggaggaccaggacatgaagaacccatccccatgtcaacatatgggtggaatctagtgcgtctgcaaagtggagttgacgttttcttcaccccgccagaaaagtgtgatacattgttgtgtgacataggggagtcgtcaccaaatcccacgatagaagcaggacgaacactcagagtcctcaacttagtggaaaattggttgaacaataacacccaattttgcataaaggtcctcaacccatatatgccttcagtcatagaaaaaatggaagcattacaaaggaaatatggaggagccttagtgaggaatccactctcacgaaactccacgcatgaaatgtactgggtatctaatgccaccgggaacatagtgtcatcagtgaacatgatttcaaggatgttgattaacagattcacaatgaaacacaagaaagccacttacgagccagatgttgacctaggaagtggaacccgcaacattggaattgaaagtgagataccaaatctagacataataggaaagagaatagagaaaataaaacaagagcatgaaacatcatggcactatgatcaagaccacccatacaaaacgtgggcttaccatggcagctatgaaacaaaacaaactggatcagcatcatctatggtgaacggagtggtcagattgctgacaaaaccttgggacgtcgtccctatggtgacacagatggcaatgacagacacgactccttttggacaacagcgcgttttcaaagagaaagtagacacgagaacccaagaaccgaaggaaggcacaaagaaactgatgaaaattacggcagagtggctttggaaagaactaggaaagaaaaagacacctaggatgtgtaccagagaagaattcacaagaaaagtgagaagcaatgcagccttgggggccatattcactgatgagaacaaatggaaatcggcacgtgaggctgttgaagatggtaggttctgggagctggttgacagggaaagaaatctccatcttgaaggaaagtgtgaaacatgtgtgtacaacatgatgggaaaaagagagaagaaactaggggagttcggcaaggcaaaaggtagcagagccatatggtacatgtggcttggagcacgcttcttagagtttgaagccctaggattcctgaatgaagatcactggttctccagagggaactccctgagtggagtggaaggagaagggctgcacaggctaggctacattttaagagacgtgggcaagaaggaagggggggcaatgtacgccgatgatacagcaggatgggacacaagaatcacactagaagacttaaaaaatgaagaaatggtaacgaaccacatgaaaggagaacacaagaaactagccgaggccatattcaaactaacgtaccaaaacaaggtggtgcgtgtgcaaagaccaacaccaagaggtacagtaatggatatcatatcgagaagagaccaaagaggcagtgggcaagtcggcacctatggccttaataccttcaccaatatggaagcccaattaattagacagatggagggagaaggaatcttcaaaagcattcagcacctgacagccacagaagaaatcgctgtacagaactggctagcaagagtggggcgtgaaaggctatcaagaatggcaatcagtggagatgattgtgttgtaaaacctatagatgacagatttgcaagtgctttaacagctctaaatgacatgggaaaagttagaaaagatatacaacaatgggaaccttcaagaggatggaacgattggacacaagtgcctttctgttcacaccactttcatgagttagtcatgaaagatggtcgcgtgctcgtagtcccatgcagaaaccaagatgaactgattggtagagcccgaatttcccagggagctgggtggtctttgaaagagacggcctgtttgggaaagtcttacgcccaaatgtggactctgatgtacttccacagacgtgacctcagactggcggcaaatgccatctgctcggcagtcccgtcacattgggttccaacaagtcgaacaacctggtccatacacgctaagcatgaatggatgacgacggaagacatgctggcagtctggaacagggtgtggatccaagaaaacccgtggatggaagataaaactccagtggaatcatgggaagaagtcccatacttgggaaaaagagaagaccaatggtgcggctcattgattgggctaacaagcagggctacctgggcaaagaacatccaaacagcaataaatcaagtcagatcccttataggcaatgaggaatacacagactacatgccatccatgaagagatttagaagggaagaggaagaggcaggtgtcctgtggtagaaggcaaaactaacatgaaacaaggctaaaagtcaggtcggattaagccatagtacggaaaaaactatgctacctgtgagccccgtccaaggacgttaaaagaagtcaggccatcacaaaatgccacagcttgagtaaactgtgcagcctgtagctccacctgaggaggtgtaaaaaacctgggaggccacaaaccatggaagctgtacgcatggcgtagtggactagcggttagaggagacccctcccttacaaatcgcagcaaacaacgggggcccaaggtgagatgaagctgtaatctcactggaaggactagaggttagaggagacccccccaaaacaaaaaacagcatattgacgctgggaaagaccagagatcctgctgtctcctcagcatcattccaggcacagaacgccagaaaatggaatggtgctgttgaatcaacaggttct

SEQ ID NO: 5 - DNA, 10708 bp, Dengue virus
  source 1..10708: mol_type = genomic DNA
agttgttagtctacgtggaccgacaagaacagtttcgactcggaagcttgcttaacgtagtgctaacagttttttattagagagcagatctctgatgaacaaccaacggaagaagacgggaaaaccgtctatcaatatgctgaaacgcgtgagaaaccgtgtgtcaactggatcacagttggcgaagagattctcaaaaggactgctgaacggccagggaccaatgaaattggttatggcgttcatagctttcctcagatttctagccattccaccaacagcaggagtcttggctagatggggaaccttcaagaagtcgggggccattaaggtcctgaaaggctttaagaaggagatctcaaacatgctgagcataatcaacaaacggaaaaagacatcgctctgtctcatgatgatattgccagcagcacttgctttccacttgacttcacgagatggagagccgcgcatgattgtggggaagaatgaaagaggaaaatccctactttttaagacagcctctggaattaacatgtgcacactcatagccatggacttgggagagatgtgtgatgacacggtcacttacaaatgcccccatattaccgaagtggaacctgaagacattgactgctggtgcaacctcacatcaacatgggtgacttatggaacgtgcaatcaagccggagagcatagacgcgataagagatcagtggcgttagctccccatgtcggcatgggactggatacacgcacccaaacttggatgtcggctgaaggagcttggaggcaagtcgagaaggtagagacatgggcccttaggcacccagggttcaccatactagccctatttcttgcccattacataggcacttccttgacccagaaggtggttatttttatactgctaatgctggtcaccccatccatgacaatgagatgtgtgggagtaggaaacagagattttgtggaaggactatcaggagctacgtgggttgacgtggtgctcgagcacggggggtgtgtgaccaccatggctaagaacaagcccacgttggatatagagcttcagaagaccgaggccacccaactggcgaccctaaggaagctatgcattgaggggaaaatcaccaacataacaactgactcaagatgtcctacccaaggggaagcggttttgcctgaggagcaggaccaaaactacgtgtgtaagcatacatacgtagacagaggctgggggaacggatgtggtttgtttggtaagggaagcttggtaacatgtgcgaaatttcaatgcctggaaccaatagagggaaaagtggtgcaatatgagaacctcaaatacaccgttatcatcacagtgcacacaggagaccaacaccaggtgggaaatgaaacgcagggagtcacggctgagataacacctcaggcatcaaccactgaagccatcttgcctgaatatggaacccttgggctagaatgctcaccacggacaggtttggacttcaatgaaatgatcttgctaacaatgaagaacaaagcatggatggtacatagacaatggttttttgacctacctctaccatggacatcaggagctacaacggaaacaccaacctggaacaggaaggagcttcttgtgacatttaaaaacgcacatgcgaagaaacaagaagtagttgttcttgggtcgcaagagggagcaatgcataccgcattgacaggagccacagaaatccaaaactcaggaggcacaagcatttttgcggggcacttaaaatgtagacttaagatggacaaattagaactcaaggggatgagctatgcaatgtgcacgaatacctttgtgttgaagaaagaagtctcagaaacgcagcatgggacaatacttatcaaggtcgagtacaaaggggaagatgtaccttgcaagattcctttctccacagaggatggacaagggaaagctcacaatggcagactgattacagccaacccagtggtgactaagaaggaggagcctgtcaatattgaggctgaacctccttttggggaaagcaatatagtaattggaattggagacaacgccttgaaaatcaactggtacaagaagggaagctctattgggaagatgttcgaggccactgctagaggtgcaaggcgcatggccatcttgggagacacagcttgggactttggatcagtgggtggtgttctgaactcattaggcaaaatggtgcaccaaatattcggaagtgcttacacagccctattcagtggagtctcttgggtaatgaaaattggaataggagttctcttgacttggatagggttgaattcaaaaaacacatccatgtcattttcatgcattgcgataggaatcatcacactctatctgggagctgtggtgcaagctgacatggggtgtgttataaactggaaaggcaaagaactcaagtgtggaagtggaatcttcgtcaccaacgaggtccatacctggacagagcaatacaaattccaagcagactccccaaaaagattggcgacagccattgcaggcgcttgggagaatggagtgtgcggaattaggtcaacaaccagaatggagaatctcctgtggaagcaaatagccaatgaactgaactacatattgtgggaaaacaatatcaaattaacggttgttgtgggcgatataattggggtcttagagcaagggaaaagaacactaacaccacaacccatggagctaaaatactcatggaaaacgtggggaaaggcaaaaatagtgacagctgaaacacaaaattcttctttcataatagatggaccaaacacaccggagtgtccaagtgcctcaagagcatggaatgtgtgggaggtggaagattacgggttcggagtcttcacaaccaacatatggctgaaactccgagaggtgtatacccaactatgtgaccataggttaatgtcggcagccgtcaaggatgaaagggccgtacatgccgacatgggctattggatagaaagtcaaaagaatggaagttggaagctagaaaaagcatccctcatagaggtgaaaacctgcacatggccaaaatcacataccctttggagtaatggtgtgttagagagtgacatgatcattccaaaaagtctagctggtcctatctcgcaacacaactacaggcccgggtaccacacccagacggcgggaccttggcatttaggaaaattagagctggacttcaactattgtgaaggaacaacagttgtcatcacagaaaactgtgggacaagaggcccatcattgagaacaacaacagtgtcagggaagttaatacacgaatggtgctgccgctcgtgcacacttcctcccctgcgatacatgggagaagacggttgctggtatggcatggaaatcagacccatcagtgagaaagaagaaaacatggtaaagtctttagtctcagcgggaagtggagaggtggacaacttcacaatgggtgtcttgtgtttggcaatcctctttgaagaggtgatgagaggaaaatttgggaagaaacacatgattgcgggggttttcttcacgtttgtactccttctctcagggcaaataacatggagagatatggcgcacacactaataatgattgggtccaatgcatctgacaggatgggaatgggcgtcacctacctagctttaattgcaacatttaaaatccagccatttttggctttgggatttttcctaagaaaactgacatccagagaaaatttattgttaggagttgggctggctatggcaacaacgttacaactgccagaggacattgaacaaatggcaaatggaatcgctctggggctcatggctctcaaactgataacacaatttgaaacataccaactatggacagcattaatctccttaacgtgttcaaatacaatttttacgttgactgttgcctggagaacagccaccctgattttggctggagtttcacttttaccagtgtgccagtcttcgagtatgaggaaaacagactggcttccaatgacagtggcagctatgggagttccacctctaccactttttatttttagcttaaaagacacactcaaaaggagaagctggccactgaatgaaggggtgatggctgttgggcttgtgagcattctggccagttctctccttagaaatgatgtacccatggctggaccattagtggccgggggcttgctgatagcgtgctacgtcataactggcacgtcagcagacctcaccgtagaaaaagcagcagatgtaacatgggaggaagaggctgagcaaacaggagtgtcccacaacttaatgatcacagttgatgatgatggaacaatgagaataaaagatgatgagactgagaatatcttaacagtgcttttgaaaacagcattactaatagtgtcaggaatctttccatactccatacccgcaacattgttggtctggcatacttggcaaaagcaaacccaaagatccggcgttctatgggatgtacccagccctccagagacacagaaagcagaactggaagaaggggtctataggatcaaacagcaaggaatttttgggaaaacccaagtaggggttggagtacagaaagaaggagtctttcacaccatgtggcacgttacaagaggggcagtgttgacatataatgggaaaagactggaaccaaattgggctagcgtgaaaaaagatctgatttcatacggaggaggatggagattgagcgcacaatggcaaaagggggaggaggtgcaggttattgccgtagagcctgggaagaacccaaagaactttcaaaccatgccaggcacttttcagactacaacaggggaaataggagcaattgcactggatttcaagcccggaacttcaggatctcctatcataaacagagagggaaaggtagtgggactgtatggcaatggagtggttacaaagaatggtggctacgtcagcggaatagcgcaaacgaatgcagaaccagatggaccgacaccagaattggaagaagagatgttcaaaaagcgaaatctaaccataatggatcttcatcctgggtcaggaaagacacggaaataccttccagctattgttagagaggcaatcaagagacgtttgagaactctaattctggcaccaacaagggtggttgcagctgagatggaagaagcattgaaagggctcccaataaggtaccaaacaacagcaacaaaatctgaacacacaggaagagagattgttgatctgatgtgccacgcaacgttcacaatgcgtctgctgtcaccagttagggttccaaactataacttgataataatggatgaagcccatttcacagacccagccagtatagctgctagagggtacatatcaactcgtgttggaatgggagaagcagccgcaatattcatgacagcaacgccccctggaacagctgatgcctttccccagagcaacgctccaattcaagatgaagaaagggacataccagaacgctcatggaattcaggcaatgaatggataaccgacttcgctgggaaaacggtgtggtttgtccccagcattaaagccggaaatgacatagcaaattgcctgcggaaaaacgggaaaaaggtcattcaacttagtaggaagacttttgacacagaatatcagaaaaccaaactgaatgattgggactttgtggtgacgactgacatttcagaaatgggggccaatttcaaagcagatagagtgatcgacccaagaagatgtctcaaaccagtgatcctgacagatggaccagagcgggtgatcctggctggaccaatgccagtcaccgcagcgagtgctgcgcaaaggagagggagagttggcaggaacccacaaaaagaaaatgaccagtacatattcacgggccagcctctcaacaatgatgaagaccatgctcactggacagaagcaaaaatgctgctggacaacattaacacaccagaagggatcataccagctctctttgagccagaaagggagaagtcagccgccatagacggtgagtatcgcctgaaaggtgagtccaggaagactttcgtggaactcatgaggaggggtgaccttccagtctggttagcccataaagtagcatcagaagggatcaaatatacagatagaaaatggtgctttgatggacaacgtaataatcaaattttagaagagaacatggatgtggaaatctggacaaaggaaggagaaaagaaaaaattgagacctaggtggcttgatgctcgcacctattcagatcccttagcactcaaggaattcaaggactttgcggctggcaggaagtcaatagcccttgatcttgtgacagaaataggaagagtgccttcacacctagctcatagaacgagaaacgctctggacaatctggtgatgctgcatacgtcagaacatggcggtaaggcctacaggcatgcggtggaggaactaccagagacaatggaaacactcctactcttgggactcatgatcttgttgacaggtggagcaatgcttttcttaatatcaggtaaagggattggaaagacttcaataggactcatttgtgtaattgcttccagcggcatgttgtggatggccgaaatcccactccaatggatcgcgtcggccatagtcctggagttttttatgatggtgttgcttataccagaaccagagaagcagagaaccccccaagacaaccaactcgcatatgtcgtgataggcatacttacactggcagcaataatagcagccaatgaaatgggattgttggaaactacaaagagagatttaggaatgtctaaggagccaggtgttgtttctccaaccagctatttagatgtggacttgcacccagcatcagcctggacattgtacgctgtggccactacagtaataacaccaatgttaagacataccatagagaattccacagcaaatgtgtccttggcagctatagccaaccaggcagtggtcctgatgggtttggacaaaggatggccaatatcaaaaatggacttaggagtacccctgctggcattgggttgctattcacaagtgaacccactgactctaacagcggcagtactcttgctgatcacacattatgccattataggtccaggattgcaggcaaaagccacccgtgaagctcagaaaaggacagctgctggaataatgaagaatccaacagtggatgggataatgacaatagacctagatcctgtaatatatgattcaaaatttgaaaagcaactgggacaggttatgctcctggttttgtgtgcagttcaacttttgttaatgagaacatcatgggccttgtgtgaagctttaaccctagctacaggaccaataacaacactctgggaaggatcacctgggaagttttggaacaccacgatagctgtttccatggcgaacatttttagagggagctatttagcaggagctgggcttgctttctctattatgaaatcagttggaacagggaaaagaggaacaggctcacagggtgaaactttgggagaaaaatggaaaaagaagttaaatcaattatcccggaaagagtttgacctttacaagaaatctggaatcactgaggtggatagaacagaagccaaagaagggttgaaaagaggagaaataacacatcatgccgtgtccagaggtagtgcaaaacttcaatggtttgtggagagaaacatggtcattcccgaaggaagagttatagacttgggctgtggaagaggaggctggtcatattactgtgcaggactgaaaaaagtcacagaagtgcgaggatacacaaaaggcggtccaggacacgaagaaccagtacctatgtccacatatggatggaacatagttaagttaatgagtggaaaggatgtgttttatcttccacctgaaaagtgtgacaccctgttgtgcgacattggagaatcttcaccaagcccaacagtggaagaaagcagaactataagagttttgaagatggttgaaccatggctaaagaacaaccaattttgtattaaagtattgaacccttacatgccaactgtgattgagcacctagaaagactacaaaggaaacatggaggaatgcttgtgagaaatccactttcacgaaactccacgcacgaaatgtactggatatccaatggcacaggtaacattgtcgcttcagtcaacatggtatctagactgctactgaacaggttcacgatgacacacagaagacccaccattgagaaagatgtggatttaggagcaggaactcgacatgttaatgcggaaccagaaacacccaacatggatgtcattggggaaagaataaaaaggatcaaggaggagcataattcaacatggcactacgatgacgaaaacccctacaaaacgtgggcttaccatggatcttatgaagtcaaagccacaggctcagcctcctccatgataaatggagtcgtgaaactcctcactaaaccatgggatgtggtgcccatggtgacacagatggcaatgacagatacaactccatttggccagcagagagtctttaaagagaaagtggacaccaggacacccaggtccatgccaggaacaagaagggttatggggatcacagcggagtggctctggagaaccctgggaaggaataaaaaacccaggttatgcacaagggaagagtttacaaaaaaggtcagaactaacgcagccatgggagctgttttcacagaggagaaccaatgggacagcgcgaaagctgctgttgaggatgaggatttttggaaacttgtggacagagaacgtgaactccacaaactgggcaagtgtggaagctgtgtttacaacatgatgggtaagagagagaagaaacttggagagtttggcaaagcaaaaggcagtagagctatatggtacatgtggttgggagccaggtaccttgagttcgaagcccttggattcttaaatgaagaccactggttctcgcgtgagaactcttacagtggagtggaaggagaaggactgcacaagctaggctatatattaagggacatttccaagatacccggaggagctatgtatgctgatgacacagctggttgggacacaagaataacagaagatgacctgcacaatgaggaaaagatcacacagcaaatggaccctgaacacaggcagttagcgaacgctatatttaagctcacataccaaaacaaagtggtcaaagttcaacgaccgactccaacaggcacggtaatggatatcatatctaggaaagaccaaagaggcagtggacaggtaggaacttatggtctgaatacattcaccaacatggaagcccagttaatcagacaaatggaaggagaaggtgtgctgtcaaaggcagacctcgagaaccctcatctgccagagaagaaaattacacaatggttggaaaccaaaggagtggagaggttaaaaagaatggccataagtggggatgactgcgtggtgaaaccaatcgatgacaggttcgctaatgccctgctcgctctgaacgacatgggaaaggttcggaaagacatacctcaatggcagccatcaaagggatggcatgattggcaacaggttcctttctgctcccaccactttcatgaattgatcatgaaagatggaagaaagttggtggttccctgcagaccccaggacgaactaataggaagggcaagaatctctcaaggagcgggatggagccttagagaaaccgcatgtctggggaaagcctacgctcaaatgtggagtctcatgtattttcacagaagagacctcagactagcatccaacgccatatgttcagcagtaccagtccactgggtccccacaagtagaacgacatggtctattcacgctcaccatcagtggatgaccacagaagacatgcttactgtctggaacagagtgtggatcgaggacaatccatggatggaagacaaaactccagtcacaacctgggaaaatgttccatatctagggaagagagaagaccaatggtgcggatcacttattggtctcacttccagagcaacctgggcccagaacatacccacagcaattcaacaggttagaagccttataggcaatgaagagtttctggactacatgccttcaatgaagagatttaggaaggaggaggagtcggagggagccatttggtaaaacgtaggaagtgaaaaagaggttaactgtcaggccatattaagccacagtacggaagaagctgtgctgcctgtgagccccgtccaaggacgttaaaagaagaagtcaggccccaaagccacggtttgagcaaaccgtgctgcctgtagctccgtcgtggggacgtaaaacctgggaggctgcaaactgtggaagctgtacgcacggtgtagcagactagcggttagaggagacccctcccatgacacaacgcagcagcggggcccgagcactgagggaagctgtacctccttgcaaaggactagaggttagaggagaccccccgcaaataaaaacagcatattgacgctgggagagaccagagatcctgctgtctcctcagcatcattccaggcacagaacgccagaaaatggaatggtgctgttgaatcaacaggttct

SEQ ID NO: 6 - DNA, 10708 bp, Dengue virus
  source 1..10708: mol_type = genomic DNA
agttgttagtctacgtggaccgacaagaacagtttcgactcggaagcttgcttaacgtagtgctaacagttttttattagagagcagatctctgatgaacaaccaacggaagaagacgggaaaaccgtctatcaatatgctgaaacgcgtgagaaaccgtgtgtcaactggatcacagttggcgaagagattctcaaaaggactgctgaacggccagggaccaatgaaattggttatggcgttcatagctttcctcagatttctagccattccaccaacagcaggagtcttggctagatggggaaccttcaagaagtcgggggccattaaggtcctgaaaggctttaagaaggagatctcaaacatgctgagcataatcaacaaacggaaaaagacatcgctctgtctcatgatgatattgccagcagcacttgctttccacttgacttcacgagatggagagccgcgcatgattgtggggaagaatgaaagaggaaaatccctactttttaagacagcctctggaattaacatgtgcacactcatagccatggacttgggagagatgtgtgatgacacggtcacttacaaatgcccccatattaccgaagtggaacctgaagacattgactgctggtgcaacctcacatcaacatgggtgacttatggaacgtgcaatcaagccggagagcatagacgcgataagagatcagtggcgttagctccccatgtcggcatgggactggatacacgcacccaaacttggatgtcggctgaaggagcttggaggcaagtcgagaaggtagagacatgggcccttaggcacccagggttcaccatactagccctatttcttgcccattacataggcacttccttgacccagaaggtggttatttttatactgctaatgctggtcaccccatccatgacaatgagatgcgtgggcgtagggaatagagactttgtagagggattgagcggagcgacatgggtcgacgtcgtactcgaacacggggggtgcgtgacgactatggctaagaataagcctacactcgatatcgaactgcaaaaaaccgaagcgacacaattggcgacattgcgcaaactatgtatcgaaggtaagattacgaacattacaaccgatagtagatgccctacacaaggcgaagccgttctacctgaggagcaagaccaaaactacgtatgtaagcatacatacgttgatagggggtgggggaacggatgcggattgttcggtaaggggtcattggtcacatgcgctaagttccaatgcttagagcctatcgagggtaaggtggtacaatacgaaaaccttaagtataccgtgataattacagttcataccggagaccaacaccaagtgggaaacgagacacagggagtgacagccgaaattacgcctcaggctagtacaaccgaagcgatactacccgaatacggaacattggggttggagtgttcacctagaaccggattggactttaacgaaatgatactgttgactatgaaaaacaaggcatggatggtgcataggcaatggttttttgacctaccattgccttggactagcggagcgacaaccgaaacacctacatggaatagaaaagagctcctagtgacatttaaaaacgctcacgctaagaagcaggaagtggtcgttttagggtcacaggagggagctatgcataccgcactaaccggagcgactgagatacagaatagcggagggacatcaatcttcgccggacaccttaagtgtagattgaaaatggacaaacttgagcttaaggggatgtcatacgctatgtgtacgaacacattcgtgctgaaaaaagaggtaagcgaaacgcaacacggaacgatactgattaaggttgagtataagggcgaagacgtcccatgtaagatacctttttcgacagaggacggacagggtaaggcccataacggaagactgattaccgctaacccagtggtgaccaaaaaagaggaaccagtcaatatcgaagccgaacctccattcggagagtcaaacatagtgatagggataggcgataacgcacttaagattaactggtacaaaaaagggtcatcaatcggtaagatgtttgaggcaaccgctaggggggctagacggatggccatactcggagacaccgcatgggacttcggatccgtggggggggtacttaactcactcggtaagatggtgcaccaaattttcggatccgcatataccgctctatttagcggagtgtcatgggtgatgaaaatcggaatcggagttctattgacatggatcggattgaactctaagaatacatctatgtcattttcatgtatcgcaatcggaattattacgctatatctcggagccgtagtgcaagccgacatggggtgtgttataaactggaaaggcaaagaactcaagtgtggaagtggaatcttcgtcaccaacgaggtccatacctggacagagcaatacaaattccaagcagactccccaaaaagattggcgacagccattgcaggcgcttgggagaatggagtgtgcggaattaggtcaacaaccagaatggagaatctcctgtggaagcaaatagccaatgaactgaactacatattgtgggaaaacaatatcaaattaacggttgttgtgggcgatataattggggtcttagagcaagggaaaagaacactaacaccacaacccatggagctaaaatactcatggaaaacgtggggaaaggcaaaaatagtgacagctgaaacacaaaattcttctttcataatagatggaccaaacacaccggagtgtccaagtgcctcaagagcatggaatgtgtgggaggtggaagattacgggttcggagtcttcacaaccaacatatggctgaaactccgagaggtgtatacccaactatgtgaccataggttaatgtcggcagccgtcaaggatgaaagggccgtacatgccgacatgggctattggatagaaagtcaaaagaatggaagttggaagctagaaaaagcatccctcatagaggtgaaaacctgcacatggccaaaatcacataccctttggagtaatggtgtgttagagagtgacatgatcattccaaaaagtctagctggtcctatctcgcaacacaactacaggcccgggtaccacacccagacggcgggaccttggcatttaggaaaattagagctggacttcaactattgtgaaggaacaacagttgtcatcacagaaaactgtgggacaagaggcccatcattgagaacaacaacagtgtcagggaagttaatacacgaatggtgctgccgctcgtgcacacttcctcccctgcgatacatgggagaagacggttgctggtatggcatggaaatcagacccatcagtgagaaagaagaaaacatggtaaagtctttagtctcagcgggaagtggagaggtggacaacttcacaatgggtgtcttgtgtttggcaatcctctttgaagaggtgatgagaggaaaatttgggaagaaacacatgattgcgggggttttcttcacgtttgtactccttctctcagggcaaataacatggagagatatggcgcacacactaataatgattgggtccaatgcatctgacaggatgggaatgggcgtcacctacctagctttaattgcaacatttaaaatccagccatttttggctttgggatttttcctaagaaaactgacatccagagaaaatttattgttaggagttgggctggctatggcaacaacgttacaactgccagaggacattgaacaaatggcaaatggaatcgctctggggctcatggctctcaaactgataacacaatttgaaacataccaactatggacagcattaatctccttaacgtgttcaaatacaatttttacgttgactgttgcctggagaacagccaccctgattttggctggagtttcacttttaccagtgtgccagtcttcgagtatgaggaaaacagactggcttccaatgacagtggcagctatgggagttccacctctaccactttttatttttagcttaaaagacacactcaaaaggagaagctggccactgaatgaaggggtgatggctgttgggcttgtgagcattctggccagttctctccttagaaatgatgtacccatggctggaccattagtggccgggggcttgctgatagcgtgctacgtcataactggcacgtcagcagacctcaccgtagaaaaagcagcagatgtaacatgggaggaagaggctgagcaaacaggagtgtcccacaacttaatgatcacagttgatgatgatggaacaatgagaataaaagatgatgagactgagaatatcttaacagtgcttttgaaaacagcattactaatagtgtcaggaatctttccatactccatacccgcaacattgttggtctggcatacttggcaaaagcaaacccaaagatccggcgttctatgggatgtacccagccctccagagacacagaaagcagaactggaagaaggggtctataggatcaaacagcaaggaatttttgggaaaacccaagtaggggttggagtacagaaagaaggagtctttcacaccatgtggcacgttacaagaggggcagtgttgacatataatgggaaaagactggaaccaaattgggctagcgtgaaaaaagatctgatttcatacggaggaggatggagattgagcgcacaatggcaaaagggggaggaggtgcaggttattgccgtagagcctgggaagaacccaaagaactttcaaaccatgccaggcacttttcagactacaacaggggaaataggagcaattgcactggatttcaagcccggaacttcaggatctcctatcataaacagagagggaaaggtagtgggactgtatggcaatggagtggttacaaagaatggtggctacgtcagcggaatagcgcaaacgaatgcagaaccagatggaccgacaccagaattggaagaagagatgttcaaaaagcgaaatctaaccataatggatcttcatcctgggtcaggaaagacacggaaataccttccagctattgttagagaggcaatcaagagacgtttgagaactctaattctggcaccaacaagggtggttgcagctgagatggaagaagcattgaaagggctcccaataaggtaccaaacaacagcaacaaaatctgaacacacaggaagagagattgttgatctgatgtgccacgcaacgttcacaatgcgtctgctgtcaccagttagggttccaaactataacttgataataatggatgaagcccatttcacagacccagccagtatagctgctagagggtacatatcaactcgtgttggaatgggagaagcagccgcaatattcatgacagcaacgccccctggaacagctgatgcctttccccagagcaacgctccaattcaagatgaagaaagggacataccagaacgctcatggaattcaggcaatgaatggataaccgacttcgctgggaaaacggtgtggtttgtccccagcattaaagccggaaatgacatagcaaattgcctgcggaaaaacgggaaaaaggtcattcaacttagtaggaagacttttgacacagaatatcagaaaaccaaactgaatgattgggactttgtggtgacgactgacatttcagaaatgggggccaatttcaaagcagatagagtgatcgacccaagaagatgtctcaaaccagtgatcctgacagatggaccagagcgggtgatcctggctggaccaatgccagtcaccgcagcgagtgctgcgcaaaggagagggagagttggcaggaacccacaaaaagaaaatgaccagtacatattcacgggccagcctctcaacaatgatgaagaccatgctcactggacagaagcaaaaatgctgctggacaacattaacacaccagaagggatcataccagctctctttgagccagaaagggagaagtcagccgccatagacggtgagtatcgcctgaaaggtgagtccaggaagactttcgtggaactcatgaggaggggtgaccttccagtctggttagcccataaagtagcatcagaagggatcaaatatacagatagaaaatggtgctttgatggacaacgtaataatcaaattttagaagagaacatggatgtggaaatctggacaaaggaaggagaaaagaaaaaattgagacctaggtggcttgatgctcgcacctattcagatcccttagcactcaaggaattcaaggactttgcggctggcaggaagtcaatagcccttgatcttgtgacagaaataggaagagtgccttcacacctagctcatagaacgagaaacgctctggacaatctggtgatgctgcatacgtcagaacatggcggtaaggcctacaggcatgcggtggaggaactaccagagacaatggaaacactcctactcttgggactcatgatcttgttgacaggtggagcaatgcttttcttaatatcaggtaaagggattggaaagacttcaataggactcatttgtgtaattgcttccagcggcatgttgtggatggccgaaatcccactccaatggatcgcgtcggccatagtcctggagttttttatgatggtgttgcttataccagaaccagagaagcagagaaccccccaagacaaccaactcgcatatgtcgtgataggcatacttacactggcagcaataatagcagccaatgaaatgggattgttggaaactacaaagagagatttaggaatgtctaaggagccaggtgttgtttctccaaccagctatttagatgtggacttgcacccagcatcagcctggacattgtacgctgtggccactacagtaataacaccaatgttaagacataccatagagaattccacagcaaatgtgtccttggcagctatagccaaccaggcagtggtcctgatgggtttggacaaaggatggccaatatcaaaaatggacttaggagtacccctgctggcattgggttgctattcacaagtgaacccactgactctaacagcggcagtactcttgctgatcacacattatgccattataggtccaggattgcaggcaaaagccacccgtgaagctcagaaaaggacagctgctggaataatgaagaatccaacagtggatgggataatgacaatagacctagatcctgtaatatatgattcaaaatttgaaaagcaactgggacaggttatgctcctggttttgtgtgcagttcaacttttgttaatgagaacatcatgggccttgtgtgaagctttaaccctagctacaggaccaataacaacactctgggaaggatcacctgggaagttttggaacaccacgatagctgtttccatggcgaacatttttagagggagctatttagcaggagctgggcttgctttctctattatgaaatcagttggaacagggaaaagaggaacaggctcacagggtgaaactttgggagaaaaatggaaaaagaagttaaatcaattatcccggaaagagtttgacctttacaagaaatctggaatcactgaggtggatagaacagaagccaaagaagggttgaaaagaggagaaataacacatcatgccgtgtccagaggtagtgcaaaacttcaatggtttgtggagagaaacatggtcattcccgaaggaagagttatagacttgggctgtggaagaggaggctggtcatattactgtgcaggactgaaaaaagtcacagaagtgcgaggatacacaaaaggcggtccaggacacgaagaaccagtacctatgtccacatatggatggaacatagttaagttaatgagtggaaaggatgtgttttatcttccacctgaaaagtgtgacaccctgttgtgcgacattggagaatcttcaccaagcccaacagtggaagaaagcagaactataagagttttgaagatggttgaaccatggctaaagaacaaccaattttgtattaaagtattgaacccttacatgccaactgtgattgagcacctagaaagactacaaaggaaacatggaggaatgcttgtgagaaatccactttcacgaaactccacgcacgaaatgtactggatatccaatggcacaggtaacattgtcgcttcagtcaacatggtatctagactgctactgaacaggttcacgatgacacacagaagacccaccattgagaaagatgtggatttaggagcaggaactcgacatgttaatgcggaaccagaaacacccaacatggatgtcattggggaaagaataaaaaggatcaaggaggagcataattcaacatggcactacgatgacgaaaacccctacaaaacgtgggcttaccatggatcttatgaagtcaaagccacaggctcagcctcctccatgataaatggagtcgtgaaactcctcactaaaccatgggatgtggtgcccatggtgacacagatggcaatgacagatacaactccatttggccagcagagagtctttaaagagaaagtggacaccaggacacccaggtccatgccaggaacaagaagggttatggggatcacagcggagtggctctggagaaccctgggaaggaataaaaaacccaggttatgcacaagggaagagtttacaaaaaaggtcagaactaacgcagccatgggagctgttttcacagaggagaaccaatgggacagcgcgaaagctgctgttgaggatgaggatttttggaaacttgtggacagagaacgtgaactccacaaactgggcaagtgtggaagctgtgtttacaacatgatgggtaagagagagaagaaacttggagagtttggcaaagcaaaaggcagtagagctatatggtacatgtggttgggagccaggtaccttgagttcgaagcccttggattcttaaatgaagaccactggttctcgcgtgagaactcttacagtggagtggaaggagaaggactgcacaagctaggctatatattaagggacatttccaagatacccggaggagctatgtatgctgatgacacagctggttgggacacaagaataacagaagatgacctgcacaatgaggaaaagatcacacagcaaatggaccctgaacacaggcagttagcgaacgctatatttaagctcacataccaaaacaaagtggtcaaagttcaacgaccgactccaacaggcacggtaatggatatcatatctaggaaagaccaaagaggcagtggacaggtaggaacttatggtctgaatacattcaccaacatggaagcccagttaatcagacaaatggaaggagaaggtgtgctgtcaaaggcagacctcgagaaccctcatctgccagagaagaaaattacacaatggttggaaaccaaaggagtggagaggttaaaaagaatggccataagtggggatgactgcgtggtgaaaccaatcgatgacaggttcgctaatgccctgctcgctctgaacgacatgggaaaggttcggaaagacatacctcaatggcagccatcaaagggatggcatgattggcaacaggttcctttctgctcccaccactttcatgaattgatcatgaaagatggaagaaagttggtggttccctgcagaccccaggacgaactaataggaagggcaagaatctctcaaggagcgggatggagccttagagaaaccgcatgtctggggaaagcctacgctcaaatgtggagtctcatgtattttcacagaagagacctcagactagcatccaacgccatatgttcagcagtaccagtccactgggtccccacaagtagaacgacatggtctattcacgctcaccatcagtggatgaccacagaagacatgcttactgtctggaacagagtgtggatcgaggacaatccatggatggaagacaaaactccagtcacaacctgggaaaatgttccatatctagggaagagagaagaccaatggtgcggatcacttattggtctcacttccagagcaacctgggcccagaacatacccacagcaattcaacaggttagaagccttataggcaatgaagagtttctggactacatgccttcaatgaagagatttaggaaggaggaggagtcggagggagccatttggtaaaacgtaggaagtgaaaaagaggttaactgtcaggccatattaagccacagtacggaagaagctgtgctgcctgtgagccccgtccaaggacgttaaaagaagaagtcaggccccaaagccacggtttgagcaaaccgtgctgcctgtagctccgtcgtggggacgtaaaacctgggaggctgcaaactgtggaagctgtacgcacggtgtagcagactagcggttagaggagacccctcccatgacacaacgcagcagcggggcccgagcactgagggaagctgtacctccttgcaaaggactagaggttagaggagaccccccgcaaataaaaacagcatattgacgctgggagagaccagagatcctgctgtctcctcagcatcattccaggcacagaacgccagaaaatggaatggtgctgttgaatcaacaggttct

SEQ ID NO: 7 - DNA, 10649 bp, Dengue virus
  source 1..10649: mol_type = genomic DNA
agttgttagtctgtgtggaccgacaaggacagttccaaatcggaagcttgcttaacacagttctaacagtttgtttaaatagagagcagatctctggaaaaatgaaccaacgaaaaaaggtggttagaccacctttcaatatgctgaaacgcgagagaaaccgcgtatcaacccctcaagggttggtgaagagattctcaaccggacttttttctgggaaaggacccttacggatggtgctagcattcatcacgtttttgcgagtcctttccatcccaccaacagcagggattctgaagagatggggacagttgaagaaaaataaggccatcaagatactgattggattcaggaaggagataggccgcatgctgaacatcttgaacgggagaaaaaggtcaacgataacattgttgtgcttgattcccaccgtaatggcgtttcacttgtcaacaagagatggcgaacccctcatgatagtggcaaaacatgaaagggggagacctctcttgtttaagacaacagaggggatcaacaaatgcactctcattgccatggacttgggtgaaatgtgtgaggacactgtcacgtataaatgccccctactggtcaataccgaacctgaagacattgattgctggtgcaacctcacgtctacctgggtcatgtatgggacatgcacccagagcggagaacggagacgagagaagcgctcagtagctttgacaccacattcaggaatgggattggaaacaagagctgagacatggatgtcatcggaaggggcttggaagcatgctcagagagtagagagctggatactcagaaacccaggatttgcgctcttggcaggatttatggcttatatgattgggcaaacaggaatccagcgaactgtcttctttgtcctaatgatgctggtcgccccatcctacggaatgcggtgcgtaggagtaggaaacagagactttgtggaaggagtctcaggtggagcatgggtcgacctggtgctagaacatggaggatgcgtcacaaccatggcccagggaaaaccaaccttggattttgaactgactaagacaacagctaaggaagtggctctgttaagaacctattgcattgaagcctcaatatcaaacataactacggcaacaagatgtccaacgcaaggagagccttatctgaaagaggaacaggaccaacagtacatctgccggagagatgtggtagacagaggatggggcaatggctgtggcttgtttggaaaaggaggagttgtgacatgtgcgaagttttcatgttcggggaagataacaggcaatctggtccaaattgagaaccttgaatacacagtggttgtaacagtccacaatggagacacccatgcagtaggaaatgacacatccaatcatggagttacagccacgataactcccaggtcaccatcggtagaagtcaaattgccggactatggagaactaacactcgattgtgaacccaggtctggaattgactttaatgagatgatcctaatgaaaatgaaaaagaaaacatggctcgtgcataagcaatggtttttggatctgcctcttccatggacagcaggagcagacacatcagaggttcactggaattacaaagagagaatggtgacgttcaaggttcctcatgccaagagacaggatgtgacagtgctgggatctcaggaaggagccatgcattctgccctcgctggagccacagaagtggactccggtgatggaaatcacatgtttgcaggacatctcaagtgcaaagtccgtatggagaaattgagaatcaagggaatgtcatacacgatgtgttcaggaaagttttcaattgacaaagagatggcagaaacacagcatgggacaacagtggtgaaagtcaagtatgaaggtgctggagctccgtgtaaagtccccatagagataagagatgtaaacaaggaaaaagtggttgggcgcgttatctcatccacccctttggctgagaataccaacagtgtaaccaacatagaattagaacccccctttggggacagctacattgtgataggtgttggaaacagcgcattaacactccattggttcaggaaagggagttccattggcaagatgtttgagtccacatacagaggtgcaaaacgaatggccattctaggtgaaacagcttgggattttggttccgttggtggactgttcacatcattgggaaaggctgtacaccaggtttttggaagcgtgtatacaaccatgtttggaggagtctcatggatgattagaatcctaattgggttcttagtgttgtggattggcacgaattcaaggaacacttcaatggccatgacgtgcatagctgttggaggaattactctgtttttgggcttcacagttcaagcggacatgggttgtgtggtgtcatggagtgggagagaattgaagtgtggaagcggaatttttgtggttgacaacgtgcacacttggacagaacagtacaaattccaaccagagtccccagcgagactagcgtctgcaatattaaatgcccacaaagatggggtctgtggaattagatcaaccacgaggctggaaaatgttatgtggaagcaaataaccaatgagctaaactatgttctctgggaaggaggacatgatctcactgtagtggctggggatgtgaaaggggtgttgaccaagggcaagagagcactcacacccccagcgagtgatctgaaatattcatggaagacatgggggaaagcaaaaatcttcacccctgaagcaagaaacagcacatttttaatagacggaccagacacctctgaatgccccaatgaacgaagggcatggaattcttttgaggtggaagactatggatttggcatgttcacgaccaacatatggatgaaattccgagaaggaagttcagaagtgtgtgaccacaggttaatgtcagctgcaattaaagaccagaaagctgtgcatgctgacatgggttattggatagagagctcaaaaaaccagacctggcagatagagagagcatctcttattgaagtgaaaacatgtctgtggcccaagacccatacactgtggagcaatggagtgctggaaagccagatgcttattccaaaatcatatgcaggccctttttcacagcacaattaccgccagggctatgctacgcaaaccgtgggtccatggcacttaggcaaactagagatagactttggagaatgccccggaacaacagtcacaattcaggagaattgtgaccatagaggcccatctttgaggaccaccactgcatctggaaaactagtcacgcaatggtgttgccgctcctgcacgatgccccccttaaggttcttaggagaagatgggtgctggtatgggatggagattaggcccttgagtgaaaaagaagagaacatggtcaaatcacaggtgacggccggacagggcacatcggaaactttttcaatgggtctgttgtgcctgaccttgtttgtggaagaatgcttgaggagaagagtcaccaggaaacacatgatattagctgtggtaatcactctttgtgctatcatcctggggggcctcacatggatggacttgctacgagccctcatcatgttgggggacactatgtctggtagaataggaggacagacccacctagccatcatggcagtgttcaagatgtcaccgggatacgtgctgggtgtgtttttaaggaaactcacttcaagagagacagcactaatggtaataggaatggccatgacaacaacactttcaattccacatgacctcatggaactcattgatggaatatcactaggactaattttgctaaaaatagtaacacagtttgacaacacccaagtgggaaccttagctctttccttgactttcataagatcaacaatgtcattggtcatggcttggaggaccattatggctgtgttgtttgtggtcacactcattcctttgtgcaggacaagctgtcttcaaaaacagtctcattgggtagaaataacagcactcatcctaggagcccaagctctgccagtgtacctaatgactcttatgaaaggagcctcaagaagatcttggcctcttaacgaaggcataatggctgtgggtttggttagtctcttaggaagcgctcttttaaagaatgatgtccctttagctggcccaatggtggcaggaggcttacttctggcggcttacgtaatgagtggcagctcagcagatctgtcactagagaaggccgctaatgtgcagtgggatgaaatggcagacataacaggctcaagtccaatcatagaagtgaagcaagatgaggatggctctttctccatacgggacgtcgaggaaaccaatatgataacccttttggtgaaactggcactgataacggtgtcaggtctctaccccttggcaattccaatcacaatgaccttatggtacatgtggcaagtgaaaacacaaagatcaggagccctgtgggacgtcccttcacccgccgccactcaaaaagccgcactgtctgaaggagtgtacaggatcatgcaaagagggttattcgggaaaactcaggttggagtagggatacacatggaaggtgtatttcacacaatgtggcatgttacaagaggatcggtgatctgccacgagactgggagattggagccatcttgggctgatgtcaggaatgacatgatatcatacggtgggggatggaggcttggagataaatgggacaaagaagaagacgttcaggtcctcgctatagaaccagggaaaaatcccaaacatgtccaaacgaaacctggccttttcaagaccctaactggagaaattggagcagtaacattagatttcaaacccggaacgtctggttctcccattatcaacaggaaaggaaaagtcatcggactctatggaaatggagtggtcaccaaatcaggtgattacgtcagtgccataacacaagccgaaagaattggagagccagattatgaagtggatgaggacatttttcgaaagaaaagactaactataatggacttacaccccggagccggaaagacaaaaagaattcttccatcaatagtgagagaagccttaaaaaggaggctgcgaactttgattttggctcccacgagagtggtggcggccgagatggaagaggccctacgtggactgccaatccgttaccaaaccccagctgtaaaatcagaacacacaggaagagagattgtagacctcatgtgccatgcaaccttcacaacaagacttttgtcatcaaccagagttccaaactacaaccttatagtaatggatgaagcacatttcaccgatccttccagtgtcgcggctagaggatacatttcgaccagggtggaaatgggagaggcagcagccatcttcatgaccgcaacccctcccggagcgacagatccctttccccagagcaacagcccaatagaagacatcgagagagagattccggaaaggtcatggaacacagggttcgactggataacagactaccaagggaaaactgtgtggtttgttcccagcataaaagctggaaatgacattgcaaattgtttgagaaagtcgggaaagaaagttatccagttgagtaggaaaacctttgatacagaatatccaaaaacgaaactcacggactgggactttgtggtcactacagacatatctgaaatgggggctaactttagagctgggagagtgatagaccctagaagatgcctcaagccagttatcctaacagatgggccagagagagtcatcttagcaggtcctattccagtgactccagcaagcgctgctcagagaagagggcgaataggaaggaacccagcacaagaagacgaccaatacgttttctccggagacccactaaaaaatgatgaagaccatgcccactggacagaagcaaagatgctgcttgacaatatctacaccccagaagggatcattccaacattgtttggtccggaaagggaaaaaacccaagctattgatggagagtttcgcctcagaggggaacaaaggaagacttttgtggaattaatgaggagaggagaccttccggtgtggctgagttataaggtagcttctgctggcatttcttacaaagatcgggaatggtgctttactggggaaagaaataaccaaattttagaagaaaacatggaggttgaaatttggactagagagggagaaaagaaaaaactgaggccaaaatggttagatgcacgtgtatacgctgaccccatggctttgaaggatttcaaggagtttgccagtggaaggaagagtataactctcgacatcctaacagagatcgccagtttgccaacttacctttcctctagggccaagctcgcccttgacaacatagttatgctccacacaacagaaagaggagggagggcctatcaacatgccctgaacgaacttccggagtcactggaaacactcatgcttgtagccttactaggagctatgacagcaggtatcttcctgtttttcatgcaagggaaaggaatagggaaattgtcaatgggtttgataaccattgcggtggctagtggcttgctctgggtagcagaaattcaaccccagtggatagcggcctcaatcatactggagttttttctcatggtactgttgataccagaaccagaaaaacaaaggaccccacaagacaatcaattgatctacgtcatattgaccattctcaccattattggtctaatagcagccaacgagatggggctgatagaaaaaacaaaaacggattttgggttttaccaggtaaaaacagaaaccaccatcctcgatgtggacctgagaccagcttcagcatggacgctctatgcggtagccaccacaattctgactcccatgctgagacacaccatagaaaatacgtcggccaacctatctttagcagccatcgccaaccaggcagccgtcctaatggggcttggaaaaggatggccactccacagaatggacctcggtgtgccgctgttagcaatgggatgctattctcaagtgaacccaacaaccttgacagcatccttagtcatgcttttagtccattatgcaataataggcccaggattgcaggcaaaagccacaagagaggcccagaaaaggacagctgctggaatcatgaaaaatcccacagtggacgggataacagtgatagatctagaaccaatatcctatgacccaaaatttgaaaagcaattagggcaggtcatgttactcgtcttgtgtgctggacaactactcttgatgagaacaacatgggctttctgtgaagttttgactttggccacaggaccaatcttgaccttgtgggagggcaacccgggaaggttttggaacacgaccatagccgtatctaccgccaacattttcaggggaagttatttggcaggagctggactggctttttcactcataaagaatgcacaaacccccaggaggggaactgggaccacaggagagacactgggagagaagtggaagagacagctaaactcattagacaggaaagagtttgaagagtataaaagaagtggaatactagaagtggacaggactgaagccaagtccgccctgaaagatgggtctaaaatcaagcatgcagtatctagagggtccagtaagatcagatggattgttgagagagggatggtaaagccaaaggggaaagttgtagatcttggctgtgggagaggaggatggtcttattacatggcgacactcaagaacgtgactgaagtgaaagggtatacaaaaggaggtccaggacatgaagaaccgattcccatggctacttatggctggaatttggtcaaactccattcaggggttgacgtgttctacaaacccacagagcaagtggacaccctgctctgtgatattggggagtcatcttctaatccaacaatagaggaaggaagaacattaagagttttgaagatggtggagccatggctctcttcaaaacctgaattctgcatcaaagtcctcaacccctacatgccaacagtcatagaggagctggagaaactgcagagaaaacacggtgggaaccttgtcagatgcccgctgtccaggaactccacccatgagatgtattgggtgtcaggagcgtcgggaaatattgtgagctctgtgaacacaacatcaaagatgttgttgaacaggttcacaacaaggcataggaaacccacttatgagaaggacgtagatcttggggcaggaacgagaagtgtctctactgaaacagaaaaaccagacatgacaatcattgggagaaggcttcagcgattgcaagaggagcacaaagaaacatggcattatgatcaggaaaacccatacagaacctgggcgtatcatggaagctatgaagctccttcgacaggctctgcatcctccatggtgaacggggtggtgaaactgctaacaaaaccctgggatgtgattccaatggtgactcagttagccatgacagatacaaccccttttgggcaacaaagagtgttcaaagagaaggtggataccagaacgccgcaaccaaaaccaggcacacgaatggttatgaccacgacagccaattggctatgggccctccttggaaagaagaaaaatcccagactgtgtacaagggaagagttcatctcaaaagttagatcaaacgcagccataggcgcagtctttcaggaagaacaaggatggacatcagccagtgaagctgtgaatgacagccggttttgggaactggttgacaaagaaagggcccttcaccaggaagggaaatgtgaatcgtgtgtctataacatgatgggaaaacgtgagaaaaagttaggagagtttggcagagccaagggaagccgagcaatctggtacatgtggctgggagcgcggtttctggaatttgaagccctgggttttttgaatgaagatcactggtttggcagagaaaattcatggagtggagtggaaggggaaggtctgcacagattgggatacatcctggaggagatagacaagaaggatggagacctaatgtatgctgatgacacagcaggttgggacacaagaatcactgaggatgaccttcaaaatgaggaactgatcacggaacagatggctccccaccacaagatcctagccaaagccattttcaaactaacctatcaaaacaaagtggtgaaagtcctcagacccacaccgagaggagcggtgatggatatcatatccaggaaagaccaaagaggtagtggacaagttggaacatatggtttgaacacattcaccaacatggaagttcaactcatccgccaaatggaagctgaaggagtcatcacacaagatgacatgcagaacccaaaagggttgaaagaaagagttgagaaatggctgagagagtgtggtgtcgacaggttaaagaggatggcaatcagtggagacgattgcgtggtgaagcccctagatgagaggtttggcacttccctcctcttcttgaacgacatgggaaaggtgaggaaagacattccgcagtgggaaccatctaagggatggaaaaactggcaagaggttcctttttgctcccatcactttcacaagatctttatgaaggatggccgctcactagttgttccatgtagaaaccaggatgaactgatagggagagccagaatctcgcagggggctggatggagcttaagagaaacagcctgcctgggcaaagcttacgcccagatgtggtcgcttatgtacttccacagaagggatctgcgtttagcctccatggccatatgctcagcagttccaacggaatggtttccaacaagcagaacaacatggtcaatccatgctcatcaccaatggatgaccactgaagacatgctcaaagtgtggaacagagtgtggatagaagacaaccccaatatgattgacaagactccagtccattcgtgggaagatataccttacctagggaaaagagaggatttgtggtgtggatccctgattggactttcttctagagccacctgggcgaagaacattcacacggccataactcaggtcaggaacttgatcggaaaagaggaatacgtggattacatgccagtaatgaaaagatacagtgctccttcagagagtgaaggagttctgtaattaccaacaacaaacaccaaaggctattgaagtcaggccacttgtgccacggtttgagcaaaccgtgctgcctgtagctccgccaataatgggaggcgtaataatccctagggaggccatgcgccacggaagctgtacgcgtggcatattggactagcggttagaggagacccctcccatcactgacaaaacgcagcaaaagggggcccgaagccaggaggaagctgtactcctggtggaaggactagaggttagaggagacccccccaacacaaaaacagcatattgacgctgggaaagaccagagatcctgctgtctctacaacatcaatccaggcacagagcgccgcaagatggattggtgttgttgatccaacaggttct

SEQ ID NO: 8 - DNA, 10649 bp, Dengue virus
  source 1..10649: mol_type = genomic DNA
agttgttagtctgtgtggaccgacaaggacagttccaaatcggaagcttgcttaacacagttctaacagtttgtttaaatagagagcagatctctggaaaaatgaaccaacgaaaaaaggtggttagaccacctttcaatatgctgaaacgcgagagaaaccgcgtatcaacccctcaagggttggtgaagagattctcaaccggacttttttctgggaaaggacccttacggatggtgctagcattcatcacgtttttgcgagtcctttccatcccaccaacagcagggattctgaagagatggggacagttgaagaaaaataaggccatcaagatactgattggattcaggaaggagataggccgcatgctgaacatcttgaacgggagaaaaaggtcaacgataacattgttgtgcttgattcccaccgtaatggcgtttcacttgtcaacaagagatggcgaacccctcatgatagtggcaaaacatgaaagggggagacctctcttgtttaagacaacagaggggatcaacaaatgcactctcattgccatggacttgggtgaaatgtgtgaggacactgtcacgtataaatgccccctactggtcaataccgaacctgaagacattgattgctggtgcaacctcacgtctacctgggtcatgtatgggacatgcacccagagcggagaacggagacgagagaagcgctcagtagctttgacaccacattcaggaatgggattggaaacaagagctgagacatggatgtcatcggaaggggcttggaagcatgctcagagagtagagagctggatactcagaaacccaggatttgcgctcttggcaggatttatggcttatatgattgggcaaacaggaatccagcgaactgtcttctttgtcctaatgatgctggtcgccccatcctacggaatgagatgcgtaggcgtaggtaatcgcgatttcgttgagggagtgtcaggcggagcatgggtcgatctggtactcgaacacggaggatgcgttacgactatggcacagggaaaaccgacattggactttgagttgactaagacaaccgctaaagaggtcgcactattgcgaacatactgtatcgaagcgtcaatttcgaatattacaaccgctactaggtgtcctacacagggcgaaccataccttaaagaggaacaggaccaacagtatatttgtagaagagacgtagtcgatagggggtggggaaacggatgcggattgttcggtaaggggggagtcgttacatgcgctaagttctcatgttccggtaagattaccggtaacttagtgcaaattgagaatctcgaatataccgtagtcgttacagtgcataacggagacacacacgcagtcggaaacgatacatctaaccatggcgtaaccgctacaattacacctaggtcaccatccgttgaggttaagttgcccgattacggcgaactgacactcgattgcgaacctagatccggaatagactttaacgaaatgatactgatgaaaatgaaaaaaaagacatggttagtgcataagcaatggtttctcgacttacccctaccttggaccgccggagccgatactagcgaagtgcactggaattacaaagagagaatggttacatttaaagtgccacacgctaagagacaggacgttacagtgttagggtcacaggagggagctatgcatagcgcactagccggagcaaccgaagtcgatagcggagacggaaatcatatgttcgccggacatctgaaatgcaaagtgagaatggagaaattgcggattaagggaatgtcatacactatgtgttccggtaagttttcgattgacaaagagatggccgaaacgcaacacggaacaacagtcgttaaggttaagtacgaaggagccggagctccgtgtaaagtgccaatcgaaattagagacgttaacaaagagaaagtggtcggaagagtgatatctagtacacccctagccgaaaatacgaattccgttacgaatatcgaactcgaacccccctttggagactcatacatagtgataggagtgggtaattccgcactcacgttgcactggttcagaaagggatcatcaatcgggaagatgttcgaatcaacatataggggagcgaaaagaatggctatattgggcgaaaccgcatgggacttcggatcagtcggaggactgtttacgagtctgggtaaggccgtacatcaggtattcggatcagtgtatacaacaatgtttggcggagtgtcatggatgatacggatactgatagggtttctagtgttgtggatcggaacgaactcacgtaatacgtctatggctatgacatgtattgccgtaggggggattacactgtttctgggatttacagtgcaagcagacatgggttgtgtggtgtcatggagtgggagagaattgaagtgtggaagcggaatttttgtggttgacaacgtgcacacttggacagaacagtacaaattccaaccagagtccccagcgagactagcgtctgcaatattaaatgcccacaaagatggggtctgtggaattagatcaaccacgaggctggaaaatgttatgtggaagcaaataaccaatgagctaaactatgttctctgggaaggaggacatgatctcactgtagtggctggggatgtgaaaggggtgttgaccaagggcaagagagcactcacacccccagcgagtgatctgaaatattcatggaagacatgggggaaagcaaaaatcttcacccctgaagcaagaaacagcacatttttaatagacggaccagacacctctgaatgccccaatgaacgaagggcatggaattcttttgaggtggaagactatggatttggcatgttcacgaccaacatatggatgaaattccgagaaggaagttcagaagtgtgtgaccacaggttaatgtcagctgcaattaaagaccagaaagctgtgcatgctgacatgggttattggatagagagctcaaaaaaccagacctggcagatagagagagcatctcttattgaagtgaaaacatgtctgtggcccaagacccatacactgtggagcaatggagtgctggaaagccagatgcttattccaaaatcatatgcaggccctttttcacagcacaattaccgccagggctatgctacgcaaaccgtgggtccatggcacttaggcaaactagagatagactttggagaatgccccggaacaacagtcacaattcaggagaattgtgaccatagaggcccatctttgaggaccaccactgcatctggaaaactagtcacgcaatggtgttgccgctcctgcacgatgccccccttaaggttcttaggagaagatgggtgctggtatgggatggagattaggcccttgagtgaaaaagaagagaacatggtcaaatcacaggtgacggccggacagggcacatcggaaactttttcaatgggtctgttgtgcctgaccttgtttgtggaagaatgcttgaggagaagagtcaccaggaaacacatgatattagctgtggtaatcactctttgtgctatcatcctggggggcctcacatggatggacttgctacgagccctcatcatgttgggggacactatgtctggtagaataggaggacagacccacctagccatcatggcagtgttcaagatgtcaccgggatacgtgctgggtgtgtttttaaggaaactcacttcaagagagacagcactaatggtaataggaatggccatgacaacaacactttcaattccacatgacctcatggaactcattgatggaatatcactaggactaattttgctaaaaatagtaacacagtttgacaacacccaagtgggaaccttagctctttccttgactttcataagatcaacaatgtcattggtcatggcttggaggaccattatggctgtgttgtttgtggtcacactcattcctttgtgcaggacaagctgtcttcaaaaacagtctcattgggtagaaataacagcactcatcctaggagcccaagctctgccagtgtacctaatgactcttatgaaaggagcctcaagaagatcttggcctcttaacgaaggcataatggctgtgggtttggttagtctcttaggaagcgctcttttaaagaatgatgtccctttagctggcccaatggtggcaggaggcttacttctggcggcttacgtaatgagtggcagctcagcagatctgtcactagagaaggccgctaatgtgcagtgggatgaaatggcagacataacaggctcaagtccaatcatagaagtgaagcaagatgaggatggctctttctccatacgggacgtcgaggaaaccaatatgataacccttttggtgaaactggcactgataacggtgtcaggtctctaccccttggcaattccaatcacaatgaccttatggtacatgtggcaagtgaaaacacaaagatcaggagccctgtgggacgtcccttcacccgccgccactcaaaaagccgcactgtctgaaggagtgtacaggatcatgcaaagagggttattcgggaaaactcaggttggagtagggatacacatggaaggtgtatttcacacaatgtggcatgttacaagaggatcggtgatctgccacgagactgggagattggagccatcttgggctgatgtcaggaatgacatgatatcatacggtgggggatggaggcttggagataaatgggacaaagaagaagacgttcaggtcctcgctatagaaccagggaaaaatcccaaacatgtccaaacgaaacctggccttttcaagaccctaactggagaaattggagcagtaacattagatttcaaacccggaacgtctggttctcccattatcaacaggaaaggaaaagtcatcggactctatggaaatggagtggtcaccaaatcaggtgattacgtcagtgccataacacaagccgaaagaattggagagccagattatgaagtggatgaggacatttttcgaaagaaaagactaactataatggacttacaccccggagccggaaagacaaaaagaattcttccatcaatagtgagagaagccttaaaaaggaggctgcgaactttgattttggctcccacgagagtggtggcggccgagatggaagaggccctacgtggactgccaatccgttaccaaaccccagctgtaaaatcagaacacacaggaagagagattgtagacctcatgtgccatgcaaccttcacaacaagacttttgtcatcaaccagagttccaaactacaaccttatagtaatggatgaagcacatttcaccgatccttccagtgtcgcggctagaggatacatttcgaccagggtggaaatgggagaggcagcagccatcttcatgaccgcaacccctcccggagcgacagatccctttccccagagcaacagcccaatagaagacatcgagagagagattccggaaaggtcatggaacacagggttcgactggataacagactaccaagggaaaactgtgtggtttgttcccagcataaaagctggaaatgacattgcaaattgtttgagaaagtcgggaaagaaagttatccagttgagtaggaaaacctttgatacagaatatccaaaaacgaaactcacggactgggactttgtggtcactacagacatatctgaaatgggggctaactttagagctgggagagtgatagaccctagaagatgcctcaagccagttatcctaacagatgggccagagagagtcatcttagcaggtcctattccagtgactccagcaagcgctgctcagagaagagggcgaataggaaggaacccagcacaagaagacgaccaatacgttttctccggagacccactaaaaaatgatgaagaccatgcccactggacagaagcaaagatgctgcttgacaatatctacaccccagaagggatcattccaacattgtttggtccggaaagggaaaaaacccaagctattgatggagagtttcgcctcagaggggaacaaaggaagacttttgtggaattaatgaggagaggagaccttccggtgtggctgagttataaggtagcttctgctggcatttcttacaaagatcgggaatggtgctttactggggaaagaaataaccaaattttagaagaaaacatggaggttgaaatttggactagagagggagaaaagaaaaaactgaggccaaaatggttagatgcacgtgtatacgctgaccccatggctttgaaggatttcaaggagtttgccagtggaaggaagagtataactctcgacatcctaacagagatcgccagtttgccaacttacctttcctctagggccaagctcgcccttgacaacatagttatgctccacacaacagaaagaggagggagggcctatcaacatgccctgaacgaacttccggagtcactggaaacactcatgcttgtagccttactaggagctatgacagcaggtatcttcctgtttttcatgcaagggaaaggaatagggaaattgtcaatgggtttgataaccattgcggtggctagtggcttgctctgggtagcagaaattcaaccccagtggatagcggcctcaatcatactggagttttttctcatggtactgttgataccagaaccagaaaaacaaaggaccccacaagacaatcaattgatctacgtcatattgaccattctcaccattattggtctaatagcagccaacgagatggggctgatagaaaaaacaaaaacggattttgggttttaccaggtaaaaacagaaaccaccatcctcgatgtggacctgagaccagcttcagcatggacgctctatgcggtagccaccacaattctgactcccatgctgagacacaccatagaaaatacgtcggccaacctatctttagcagccatcgccaaccaggcagccgtcctaatggggcttggaaaaggatggccactccacagaatggacctcggtgtgccgctgttagcaatgggatgctattctcaagtgaacccaacaaccttgacagcatccttagtcatgcttttagtccattatgcaataataggcccaggattgcaggcaaaagccacaagagaggcccagaaaaggacagctgctggaatcatgaaaaatcccacagtggacgggataacagtgatagatctagaaccaatatcctatgacccaaaatttgaaaagcaattagggcaggtcatgttactcgtcttgtgtgctggacaactactcttgatgagaacaacatgggctttctgtgaagttttgactttggccacaggaccaatcttgaccttgtgggagggcaacccgggaaggttttggaacacgaccatagccgtatctaccgccaacattttcaggggaagttatttggcaggagctggactggctttttcactcataaagaatgcacaaacccccaggaggggaactgggaccacaggagagacactgggagagaagtggaagagacagctaaactcattagacaggaaagagtttgaagagtataaaagaagtggaatactagaagtggacaggactgaagccaagtccgccctgaaagatgggtctaaaatcaagcatgcagtatctagagggtccagtaagatcagatggattgttgagagagggatggtaaagccaaaggggaaagttgtagatcttggctgtgggagaggaggatggtcttattacatggcgacactcaagaacgtgactgaagtgaaagggtatacaaaaggaggtccaggacatgaagaaccgattcccatggctacttatggctggaatttggtcaaactccattcaggggttgacgtgttctacaaacccacagagcaagtggacaccctgctctgtgatattggggagtcatcttctaatccaacaatagaggaaggaagaacattaagagttttgaagatggtggagccatggctctcttcaaaacctgaattctgcatcaaagtcctcaacccctacatgccaacagtcatagaggagctggagaaactgcagagaaaacacggtgggaaccttgtcagatgcccgctgtccaggaactccacccatgagatgtattgggtgtcaggagcgtcgggaaatattgtgagctctgtgaacacaacatcaaagatgttgttgaacaggttcacaacaaggcataggaaacccacttatgagaaggacgtagatcttggggcaggaacgagaagtgtctctactgaaacagaaaaaccagacatgacaatcattgggagaaggcttcagcgattgcaagaggagcacaaagaaacatggcattatgatcaggaaaacccatacagaacctgggcgtatcatggaagctatgaagctccttcgacaggctctgcatcctccatggtgaacggggtggtgaaactgctaacaaaaccctgggatgtgattccaatggtgactcagttagccatgacagatacaaccccttttgggcaacaaagagtgttcaaagagaaggtggataccagaacgccgcaaccaaaaccaggcacacgaatggttatgaccacgacagccaattggctatgggccctccttggaaagaagaaaaatcccagactgtgtacaagggaagagttcatctcaaaagttagatcaaacgcagccataggcgcagtctttcaggaagaacaaggatggacatcagccagtgaagctgtgaatgacagccggttttgggaactggttgacaaagaaagggcccttcaccaggaagggaaatgtgaatcgtgtgtctataacatgatgggaaaacgtgagaaaaagttaggagagtttggcagagccaagggaagccgagcaatctggtacatgtggctgggagcgcggtttctggaatttgaagccctgggttttttgaatgaagatcactggtttggcagagaaaattcatggagtggagtggaaggggaaggtctgcacagattgggatacatcctggaggagatagacaagaaggatggagacctaatgtatgctgatgacacagcaggttgggacacaagaatcactgaggatgaccttcaaaatgaggaactgatcacggaacagatggctccccaccacaagatcctagccaaagccattttcaaactaacctatcaaaacaaagtggtgaaagtcctcagacccacaccgagaggagcggtgatggatatcatatccaggaaagaccaaagaggtagtggacaagttggaacatatggtttgaacacattcaccaacatggaagttcaactcatccgccaaatggaagctgaaggagtcatcacacaagatgacatgcagaacccaaaagggttgaaagaaagagttgagaaatggctgagagagtgtggtgtcgacaggttaaagaggatggcaatcagtggagacgattgcgtggtgaagcccctagatgagaggtttggcacttccctcctcttcttgaacgacatgggaaaggtgaggaaagacattccgcagtgggaaccatctaagggatggaaaaactggcaagaggttcctttttgctcccatcactttcacaagatctttatgaaggatggccgctcactagttgttccatgtagaaaccaggatgaactgatagggagagccagaatctcgcagggggctggatggagcttaagagaaacagcctgcctgggcaaagcttacgcccagatgtggtcgcttatgtacttccacagaagggatctgcgtttagcctccatggccatatgctcagcagttccaacggaatggtttccaacaagcagaacaacatggtcaatccatgctcatcaccaatggatgaccactgaagacatgctcaaagtgtggaacagagtgtggatagaagacaaccccaatatgattgacaagactccagtccattcgtgggaagatataccttacctagggaaaagagaggatttgtggtgtggatccctgattggactttcttctagagccacctgggcgaagaacattcacacggccataactcaggtcaggaacttgatcggaaaagaggaatacgtggattacatgccagtaatgaaaagatacagtgctccttcagagagtgaaggagttctgtaattaccaacaacaaacaccaaaggctattgaagtcaggccacttgtgccacggtttgagcaaaccgtgctgcctgtagctccgccaataatgggaggcgtaataatccctagggaggccatgcgccacggaagctgtacgcgtggcatattggactagcggttagaggagacccctcccatcactgacaaaacgcagcaaaagggggcccgaagccaggaggaagctgtactcctggtggaaggactagaggttagaggagacccccccaacacaaaaacagcatattgacgctgggaaagaccagagatcctgctgtctctacaacatcaatccaggcacagagcgccgcaagatggattggtgttgttgatccaacaggttct

SEQ ID NO: 9 - DNA, 10735 bp, Dengue virus
  source 1..10735: mol_type = genomic DNA
agttgttagtctacgtggaccgacaagaacagtttcgaatcggaagcttgcttaacgtagttctaacagttttttattagagagcagatctctgatgaacaaccaacggaaaaagacggctcgaccgtctttcaatatgctgaaacgcgcgagaaaccgcgtgtcaactgtttcacagttggcgaagagattctcaaaaggattgctctcaggccaaggacccatgaaattggtgatggctttcatagcattcctaagatttctagccatacccccaacagcaggaattttggctagatggggttcattcaagaagagtggagcgatcaaagtgctacggggtttcaagaaagaaatctcaaacatgttgaatataatgaatagaaggaaaagatctgtgaccatgctccttatgctgatgcctacagccttggcgttccatttgactacacgagggggagagccgcacatgatagtcagcaagcaggaaagaggaaagtcactcttgtttaagacctcagcaggtgtcaacatgtgcacccttatagcgatggatttgggagagttatgtgaggacacaatgacttacaaatgccctcgaatcactgaaactgaaccagatgacgttgattgttggtgtaatgccacagacacatgggtgacctatggaacatgttcccaaactggcgagcaccgacgagacaaacgttccgtcgcactggccccacacgtgggacttggtttggaaacaagaaccgaaacgtggatgtcctctgaaggcgcttggaaacagatacaaagagtggagacttgggccctgagacacccaggattcacggtgatagccctttttctagcacatgccataggaacatccatcacccagaaagggattattttcattttgttaatgctggtaacaccatccatggccatgcgatgcgtgggaataggcagcagggacttcgtggaaggactgtcaggagcaacttgggtagatgtggtactggaacatggaagttgcgtcaccaccatggcaaaagacaaaccaacattggacattgaactcttgaagacggaagtcacaaaccctgccgtcctgcgcaaactgtgcattgaagctaaaatatcaaacaccaccaccgactcaagatgtccaacacaaggagaagccacactagtggaagaacaagacgcgaactttgtgtgtcgacgaacgtttgtggacagaggctggggcaatggctgtggcctcttcggaaaaggaagcctaataacgtgtgcaaagttcaagtgtgtgacaaaactggaaggaaagatagttcaatatgagaacttgaaatattcagtaatagtcaccgttcacaccggagaccagcatcaagtgggaaatgaaagcacagaacatgggacaactgcaactataacacctcaagctcctacgacggaaatacagctgaccgactacggagctcttacattggattgttcacctagaacaggactagactttaatgaaatggtgttgttgacaatgaaagaaaaatcatggctagtccacaaacaatggtttttagacctaccactgccttggacctcgggagcttcaacatcacaagagacttggaacagacaagatttgctggtgacatttaagacagctcatgcaaagaagcaggaagtagtagtgttagggtcacaagagggagcaatgcataccgcactaaccggagcaaccgaaatacagactagcggaactacaacgatttttgccggtcacctgaaatgtagactgaagatggacaaactgacacttaaaggaatgtcatacgttatgtgtacgggatcctttaagctcgaaaaagaggttgccgaaacgcaacacggaacagtgctagtgcaaattaaatatgagggaaccgacgcaccatgtaagataccgtttagtacgcaagacgaaaagggcgttacgcaaaacggaagactgattaccgctaaccctatcgttacagacaaagagaaacccgttaacatagaggccgaaccaccttttggcgaatcatatatagtgataggcgcaggcgaaaaagcactaaagctgtcatggttcaaaaaaggatctagcatagggaagatgttcgaagcaaccgctaggggagctagacgaatggcaatactgggagataccgcatgggacttcggatcgatagggggagtgtttactagcgtaggtaagttggtgcatcagatattcggaaccgcatacggagtgttgtttagcggagtgtcatggactatgaagatagggataggagtgctattgacatggctcggactgaattcgagatcgactagcctatctatgacatgcatagccgtcggactggttacactgtatctaggcgtaatggtgcaagcagattcaggatgtgtaattaattggaaaggtagagaactcaagtgtggaagtggcatttttgtcaccaatgaagttcacacttggacagagcaatacaaatttcaagctgactcccctaagagactatcagcagccatcgggaaggcatgggaggagggtgtgtgtggaattcgatcagcaactcgtctcgagaacatcatgtggaagcaaatatcaaatgaactgaatcacatcttacttgaaaatgatatgaaattcacagtggttgtaggagatgttgctgggatcttggctcaaggaaagaaaatgattaggccacaacccatggaatacaaatactcgtggaaaagctggggaaaggctaaaatcataggggcagatgtacagaacaccaccttcatcatcgatggcccaaacaccccagaatgccctgatgaccaaagagcatggaacatttgggaagttgaggactatggatttggaattttcacgacaaacatatggctgaaattgcgtgattcctacacccaagtgtgtgaccaccggctaatgtcagctgccatcaaggacagcaaggcagttcacgctgacatggggtactggatagaaagtgaaaagaacgagacctggaagctggcaagagcctcattcatagaagttaaaacatgtatctggccaaaatcccacactctatggagcaatggagttctggaaagtgaaatgataattccaaagatctatggaggaccaatatctcagcacaactacagaccaggatattttacacaagcagcagggccgtggcacctaggcaagttggaactggattttgatttgtgtgagggtaccacagttgttgtggatgaacattgtggaaatcgaggaccatctcttaggaccacaacagtcacaggaaagataattcatgaatggtgttgcagatcttgcacgctaccacccttacgtttcagaggagaagatgggtgctggtacggtatggaaatcagaccagtcaaggaaaaggaagaaaatctagtcaaatcaatggtctctgcagggtcaggggaagtggacagcttttcactaggactgctatgcatatcaataatgatcgaggaggtgatgagatccagatggagtagaagaatgctgatgactggaacactggctgtgttcttccttctcataatgggacaattgacatggaacgatctgatcagattatgcatcatggttggagccaacgcttccgacaggatggggatgggaacgacgtacctagccctgatggccacttttaaaatgagaccgatgttcgctgtagggctattatttcgcagactaacatccagagaagttcttcttctaacaattggattgagtctagtggcatctgtggagttaccaaattccttggaggagctgggggatggacttgcaatgggcattatgattttaaaattattgactgactttcaatcacatcagctgtgggctaccttgctgtccttgacatttatcaaaacaacgttttccttgcactacgcatggaagacaatggctatggtactgtcaattgtatctctcttccctttatgcctgtccacgacctcccaaaaaacaacatggcttccggtgctattgggatcccttggatgcaaaccactaaccatgtttcttatagcagaaaacaaaatctggggaaggagaagttggcccctcaatgaaggaatcatggctgttggaatagtcagcatcctactaagttcactcctcaaaaatgatgtaccgctagctgggccactaatagctggaggcatgctaatagcatgttatgttatatctggaagctcagccgacctatcattagagaaagcggctgaggtctcctgggaagaagaagcagaacactctggtgcctcacacaacatattagtggaagtccaagatgatggaaccatgaagataaaggatgaagagagagatgacacgctaaccattctccttaaagcaactctgttagcagtttcaggggtgtacccattatcaataccagcgacccttttcgtgtggtacttttggcagaaaaagaaacagagatctggagtgttatgggacacacccagccctccagaagtggaaagagcagttcttgatgatggtatctatagaattatgcagagaggactgttgggcaggtcccaagtaggggtaggagttttccaagaaaacgtgttccacacaatgtggcatgtcaccaggggagctgtactcatgtatcaagggaagagattggaaccgagctgggccagtgtcaaaaaagacctgatctcatatggaggaggttggaggcttcaaggatcctggaacacaggagaagaagtgcaggtgattgctgttgaaccagggaaaaaccccaaaaatgtacaaacagcgccgggcacctttaagacccctgaaggtgaagttggagccattgccctagactttaaacctggcacatctggatctcccatcgtgaacagagaaggaaaaatagtaggtctttatggaaatggagtagtgacaacaagtggaacctacgtcagtgccatagctcaagccaaagcatcacaagaagggcccctaccagagattgaagacgaggtgtttaggaaaagaaacttaacaataatggacctacatccaggatcggggaaaacaagaagatatcttccagccatagtccgtgaggccataaaaaggaagctgcgcacactaatcctggctcccacaagggttgtcgcttccgaaatggcagaggcgctcaagggaatgccaataaggtaccaaacaacagcagtgaagagtgaacatacaggaaaagagatagttgacctcatgtgtcacgccactttcaccatgcgcctcctgtctcccgtaagagttcccaattacaacatgatcatcatggatgaagcacatttcaccgatccatccagtatagcggccagagggtacatctcaacccgagtgggcatgggtgaagcagctgcaatcttcatgacagccactcccccaggatcagtggaggcctttccacagagcaacgcagttatccaagatgaggaaagagacattcctgagagatcatggaactcaggctatgagtggatcactgacttcccaggtaaaacagtttggtttgttccaagcattaaatcaggaaatgacattgccaactgcttaagaaagaatgggaaacgggtgattcaattgagcaggaaaacctttgatacagagtaccaaaaaacaaaaaacaacgactgggactacgtcgtcacaacagacatctccgaaatgggagcaaatttccgagccgacagggtgatagacccaagacggtgtctgaaaccggtaatactaaaagatggtccagagcgtgtcattttagcaggaccaatgccagtgactgtggccagtgccgctcagaggagaggaagaattggaaggaaccacaataaggaaggtgatcagtacatctacatgggacagcctttaaacaacgatgaagatcacgctcactggacagaagcaaaaatgctccttgataatataaacacaccagaagggattatcccagccctctttgagccagagagagaaaagagtgcagcaatagacggggaatacagactgcggggtgaagcaaggaaaacgtttgtggagctcatgagaagaggagatctacctgtctggctatcctacaaagttgcctcagaaggcttccagtactctgacagaagatggtgctttgacggggaaaggaacaaccaggtgttggaggagaacatggacgtggagatctggacaaaagaaggagaaagaaagaaactacgaccccgctggctggatgccagaacatactcagacccactagccctgcgcgagtttaaagagtttgcagcagggagaagaagcgtctcaggtgatttaatattagaaatagggaagcttccacaacacttgacgcaaagggcccagaatgccctggacaacctggttatgttgcacaactccgaacaaggaggcagagcctatagacatgcaatggaagaactgccagacaccatagaaacgttgatgctcctagctttgatagctgtgttaactggtggagtgacactgttcttcctatcaggaaggggcctagggaaaacatctatcggcctactctgcgtaatggcttcaagcgtactgctatggatggccagtgtggagccccattggatagcggcctccatcatactggagttcttcctgatggtgctgcttattccagagccagacagacaacgcactccgcaggacaaccagctggcatatgtggtgataggtttgttattcatgatactgacagtagcagccaatgagatgggactgctggaaaccacaaagaaagacttagggattggccatgtggctgttgaaaatcaccaccatgccgcaatgctggacgtagacttacatccagcttcagcctggaccctctatgcagtggccacaacaattatcactcccatgatgaggcacacaatcgaaaacacaacggcaaacatttccctgacagccattgcaaaccaggcagctatattgatgggacttgacaaaggatggccaatatcgaagatggacataggagttccacttctcgccttggggtgctattcccaggtgaatccactgacgctgacagcggcggtattgatgctagtggctcattacgccataattggacctggactgcaagcaaaagctactagagaagctcaaaaaaggacagcggccggaataatgaaaaatccaaccgttgatggaattgttgcaatagatttggaccctgtggtttatgatgcaaaatttgaaaaacaactaggccaaataatgttgttgatactatgcacatcacagatcctcttgatgcggactacatgggccttgtgcgagtccatcacactggccactggacctctgaccacgctttgggagggatctccaggaaaattttggaacaccacgatagcggtttccatggcaaacattttcagaggaagttatctagcaggagcaggtctggccttctcattaatgaaatctctaggaggaggtaggagaggcacgggagcccaaggggaaacactgggagagaaatggaaaagacagctgaaccaactgagcaagtcagaatttaacacctataaaaggagtgggattatggaagtggacagatccgaagccaaagagggattgaaaagaggagaaacaaccaaacatgcagtgtcgagaggaaccgctaaactgaggtggttcgtggagaggaaccttgtgaaaccagaagggaaagtcatagacctcggttgtggaagaggtggctggtcatactattgcgctgggctgaagaaagtcacagaagtgaaggggtatacaaaaggaggacctggacatgaggaaccaatcccaatggcgacctatggatggaacctagtaaagctgcactctgggaaagacgtattttttataccacctgagaaatgtgacacccttttgtgtgatattggtgagtcctctccaaacccaactatagaggaaggaagaacgctacgcgtcctaaagatggtggaaccatggctcagaggaaaccaattttgcataaaaattctgaatccctacatgccaagtgtggtggaaactctggagcaaatgcaaagaaaacatggaggaatgctagtgcgaaatccactttcaagaaattctactcatgaaatgtattgggtttcatgtggaacaggaaacattgtgtcagcagtaaacatgacatctagaatgttgctaaatcgattcacaatggctcacaggaaaccaacatatgaaagagacgtggacctaggcgccggaacaagacatgtggcagtggaaccagaggtagccaacctagatatcattggccagaggatagagaacataaaacatgaacataagtcaacatggcattatgatgaggacaatccatataaaacatgggcctatcatggatcatatgaggtcaagccatcaggatcagcctcatccatggtcaatggcgtggtgaaactgctcaccaaaccatgggatgtcatccctatggtcacacaaatagccatgactgacactacaccctttggacaacagagggtgtttaaagagaaagttgacacacgcacaccaaaagcaaaacggggcacagcacaaatcatggaggtgacagccaagtggttatggggttttctttctagaaacaagaaaccaagaatttgcacaagagaggagttcacaagaaaagttaggtcaaacgcagccattggagcagtgttcgttgatgaaaatcaatggaactcagcaaaagaagcagtggaagatgagcggttctgggaccttgtgcatagagagagggagcttcacaaacagggaaaatgtgctacgtgtgtttacaacatgatggggaagagagagaaaaagctaggagagttcggaaaggcaaaaggaagtcgtgcaatatggtacatgtggttgggagcacgctttctagagttcgaagctcttggtttcatgaacgaagatcactggttcagcagagagaattcactcagcggagtggaaggagaaggactccacaaacttggatatatactcagagacatatcaaagattccagggggaaacatgtatgcagatgacacagccggatgggatacaaggataacagaggatgaccttcagaatgaggccagaattactgacatcatggaacccgaacatgccctcctggctaagtcaatcttcaagttaacctaccaaaataaggtggtaagggtacagagaccagcaaaaaatggaaccgtgatggatgtcatatccagacgtgaccagagaggaagtggtcaggtcggaacttatggcttaaacactttcaccaacatggaagcccagctgataagacaaatggagtctgagggaatcttttcacccagcgaattagagaccccaaatttagccgagagagttctcgactggctggaaaaatatggcgtcgaaaggctgaaaagaatggcaatcagcggagatgactgcgtagtgaaaccaattgatgataggtttgcaacagccttgacagctctgaatgatatgggaaaagtaagaaaagatataccacaatgggaaccttcaaaaggatggaatgattggcaacaagtgcctttttgttcacaccacttccaccagctgattatgaaggatgggagggaaatagtggtgccatgccgcaaccaagatgaacttgtgggtagggctagagtatcacaaggtgctggatggagcctgagagaaactgcatgcctaggcaagtcatatgcacaaatgtggcagctgatgtacttccacaggagagacctgagactagccgctaatgctatctgttcagccgttccagttgattggatcccaaccagccgtaccacctggtcgatccatgcccatcaccaatggatgacaacagaagacatgctgtcagtgtggaatagggtttggatagaggaaaacccatggatggaggacaaaacccacatatccagttggggagatgttccatatttaggaaaaagggaagaccaatggtgtggatccctgataggcttaacagcaagggccacctgggccaccaacatacaagtggccataaaccaagtgagaagactaattgggaatgagaattatctagattacatgacatcaatgaagagattcaagaacgagagtgatcccgaaggggcactctggtgagtcaacacatttacaaaataaaggaaaataagaaatcaaacaaggcaagaagtcaggccggattaagccatagtacggtaagagctatgctgcctgtgagccccgtctaaggacgtaaaatgaagtcaggccgaaagccacggcttgagcaaaccgtgctgcctgtagctccatcgtggggatgtaaaaacctgggaggctgcaacccatggaagctgtacgcatggggtagcagactagtggttagaggagacccctcccgaaacataacgcagcagcggggcccaacaccaggggaagctgtaccctggtggtaaggactagaggttagaggagaccccccgcataacaataaacagcatattgacgctgggagagaccagagatcctgctgtctctacagcatcattccaggcacagaacgccagaaaatggaatggtgctgttgaatcaacaggttct

SEQ ID NO: 10 - DNA, 10724 bp, Dengue virus
  source 1..10724: mol_type = genomic DNA
agttgttagtctacgtggaccgacaaagacagattctttgagggagctaagctcaacgtagttctaacagttttttaattagagagcagatctctgatgaataaccaacgaaaaaaggcgagaagtacgcctttcaatatgctgaaacgcgagagaaaccgcgtgtcaactgtgcaacagctgacaaagagattctcacttggaatgctgcaaggacgcggaccattaaaactgttcatggcccttgtggcgttccttcgtttcctaacaatcccaccaacagcagggatactaaaaagatggggaacgatcaaaaaatcaaaagctatcaatgttttgagagggttcaggaaagagattggaaggatgctgaacatcttgaacaagagacgcaggacagcaggcgtgattgttatgttgattccaacagcgatggcgttccatttaaccacacgcaatggagaaccacacatgatcgttggtaggcaggagaaagggaaaagtcttctgttcaaaacagaggatggtgttaacatgtgtactctcatggccatagaccttggtgaattgtgtgaagatacaatcacgtacaagtgtcctctcctcagacaaaatgaaccagaagacatagattgttggtgcaactctacgtccacatgggtaacttatgggacatgtaccaccacaggagaacacagaagagaaaaaagatcagtggcgctcgttccacatgtaggtatgggactggagacacgaactgaaacatggatgtcatcagaaggggcctggaaacatgttcagagaattgaaacctggatcttgagacatccaggttttaccataatggcagcaatcctggcatacaccataggaacgacacatttccaaagggccttgattttcattttactgacagctgtcgctccttcaatgacaatgcgctgcataggaatatcaaatagagacttcgtagaaggggtttcaggaggaagctgggttgacatagtcttagaacatggaagttgtgtgacgacgatggcaaaaaacaaaccaacattggattttgaactgataaaaacagaagccaaacaacctgccactctaaggaagtactgtatagaagcaaagctgaccaacacaacaacagaatcgcgttgcccaacacaaggggaacccagtctaatgaggagcaggacaaaaggttcatctgcaaacactccatggtagacagaggatggggaaatggatgtggattatttggaaagggaggcattgtgacctgtgctatgtttacatgcaaaaagaacatggaaggaaaagtcgtgcagccagaaaatttggaatacaccatcgtgataacacctcactcaggagaggagcacgctgtaggtaatgacacaggaaagcatggcaaggaaatcaaaataacaccacagagctccatcacagaagcagaactgacaggctatggcactgtcacgatggagtgctctccgagaacgggcctcgacttcaatgagatggtactgctgcagatggaagacaaagcttggctggtgcacaggcaatggttcctagacctgccgttaccatggctacccggagcggacacacaaggatcaaattggatacagaaagagacattggtcactttcaaaaatccccacgcgaagaaacaggacgtagtcgtactcggatcacaggaaggcgcaatgcataccgcattgacaggcgctacagagatacagatgtctagcggaaatctgttgtttacagggcatctgaaatgtagactgagaatggacaaactgcaattgaagggaatgtcatactctatgtgtacgggtaagtttaagatagtcaaagagatagccgaaacacaacacggaacaatcgtaattagggtgcaatacgaaggcgacgggtcaccatgtaagataccattcgaaattacagacctcgaaaaaagacacgtactcggaagactgataacagtgaatccgatcgttacggaaaaagactcacccgttaatatcgaagccgaaccaccattcggagactcatacataataatcggagtcgaacccggacaattgaaactgaattggtttaaaaaagggtcatcaatcggacaaatgttcgaaacaactatgagaggcgctaagcgtatggctatactcggagacacagcatgggacttcggatccttagggggagtgtttacgtcaatcggtaaggcactacaccaggtattcggagcgatatacggagccgcatttagcggagtgtcgtggacaatgaagatactgatcggagtgataatcacatggatcggaatgaatagtaggtctacaagtctatccgttagcttagtgttagtcggagtcgttacactgtatctaggcgctatggtgcaagccgatagtggttgcgttgtgagctggaaaaataaagaactgaaatgtggcagcgggatcttcatcacagataacgtacacacatggacagaacaatataagttccaaccagaatccccttcaaaactagcttcagctatccaaaaagctcatgaagagggcatttgtggaatccgctcagtaacaagattggagaatctgatgtggaaacaaataacaccagaattgaatcatattctatcagaaaatgaggtaaagttgaccattatgacaggagacattagaggaatcatgcaggcaggaaaacgatccttgcggccccagcccactgagctgaagtactcatggaaaacatggggaaaggcgaaaatgctctccacagagtctcacaatcagacctttcttattgatggccctgaaacagcagaatgccccaacacaaacagagcctggaactcgctggaagttgaagactatggttttggagttttcaccaccaatatatggctgaaattgagagaaaaacaggatgtattttgtgactcaaaactcatgtcagcggccattaaagacaacagagccgttcatgctgatatgggttattggatagaaagtgcactcaatgacacatggaagatggagaaagcctccttcattgaagttaaaagctgccactggccaaagtcacacaccctttggagcaatggagtattagaaagtgagatgataatcccaaaaaattttgccgggccagtgtcacaacacaactacagaccaggctaccatacacaaacagcaggaccttggcatctaggtaagcttgagatggactttgatctctgcgaaggaactacagtggtggtgactgaggactgtggaaatagaggaccctctttaagaacgaccactgcctctggaaaactcataacagaatggtgctgccgatcctgcacactaccacctctaagatacagaggtgaggatggatgctggtacgggatggaaatcagaccattgaaagagaaagaagagaatttggtcaactccttggtcacagccggacatgggcagattgacaacttttcactaggagtcttgggaatggcactgttcctggaagaaatgctcaggacccgaataggaacgaaacatgcaatactgctagttgcagtatcttttgtgacattgattactgggaacatgtcttttagagacctgggaagagtgatggttatggtgggcgctaccatgacggatgacataggtatgggagtgacttatcttgccctactagcagcttttaaggttagaccaacttttgcagctggactactcttaagaaaactgacctccaaggaattgatgatggccaccataggaatcgcactcctttcccaaagcaccataccagagaccattcttgaactgactgatgcattagccctgggcatgatggtcctcaaaatagtgagaaatatggaaaaataccaattggcagtgactatcatggctatttcatgtgtcccaaatgcagtgatactgcaaaacgcatggaaggtgagttgcacaatattggcagcggtgtccgtttcaccactgctcttaacatcctcacagcagaaagcggattggataccactggcattgacgataaaaggtctcaatccaacagccatttttttaacaactctctcgaggaccagcaagaaaaggagctggccgctaaatgaagctatcatggcagttgggatggtgagcattttagccagttctctcctaaagaatgatattcctatgacaggtccattagtggctggaggactcctcaccgtatgttacgtgctcactggacgatcggccgatttggaactggagagagctgccgatgtaaaatgggaagatcaggcagaaatatcaggaagcagcccaatcctgtcaataacaatatcagaagatggcagcatgtcgataaaaaatgaagaggaagaacaaacactgaccatactcatcagaacgggattgttggtgatctcaggagtctttccagtatcgataccaattacggcagcagcatggtacctgtgggaagtaaagaaacaacgggctggagtactgtgggacgtcccttcacccccaccagtggaaaaagccgaactggaggatggagcctacagaatcaagcaaagagggatccttggatattctcagattggagccggagtttacaaagaaggaacattccatacaatgtggcacgtcacacgtggtgctgttctgatgcatagagggaagaggattgaaccatcatgggcagatgtcaagaaagacctaatatcatatggaggaggctggaagctagaaggagaatggaaggaaggagaggaagtccaagtcctggcattggaacctggaaaaaatccaagagccgtccaaacgaaacctggaatattcaaaaccaacaccggaaccataggcgccgtatctctggacttttcccctggaacgtcaggatctccaatcgtcgacagaaaaggaaaagttgtgggtctttacggtaatggtgttgtcacaaggagtggagcatatgtaagtgctatagcccagaccgaaaaaagcattgaagacaatccagagatcgaagatgacattttccgaaagaaaagattgaccatcatggacctccatccaggagcaggaaagacaaaaagataccttccagccatagttagagaagccataaaacgtggcttgagaacattgatcctggctcccactagagtagtggcagctgaaatggaggaagctcttagaggacttccaataagataccaaactacagccatcaaaaccgagcataccgggcgggagatcgtggacctaatgtgtcatgccacatttactatgaggctgttatcaccagtcagagtgccaaattacaacctgatcatcatggacgaagcccacttcacagacccagcaagtatagcagctagaggatacatttcaactcgagtagagatgggtgaagcagccgggattttcatgacagccactcctccgggaagtagagacccatttcctcagagcaatgcaccaattatggatgaggaaagagaaatccctgagcgttcatggaattcaggacacgaatgggtcacggattttaaggggaagactgtttggtttgttccaagtataaaagcaggaaatgatatagcagcttgtcttaggaaaaatggaaagaaagtgatacaactcagtaggaagacttttgactctgagtatgttaagactagagccaatgattgggactttgtggtcacaactgacatttcagaaatgggtgccaacttcaaggctgagagggttatagaccccagacgttgcatgaaaccagttatactaacagatggcgaggagcgggtgatcttggctggacctatgccagtgacccactctagtgcagcgcaaagaagagggagaataggaagaaatccaaaaaatgaaaatgaccagtacatatacatgggggaacctcttgaaaatgatgaagactgtgcacattggaaagaagctaaaatgctcctagataacatcaacacacctgaaggaatcattcctagtatgttcgaaccagagcgtgaaaaagtggatgccattgatggtgaataccgtttgagaggagaagcaaggaaaacctttgtggacctaatgagaagaggggacttaccagtctggttggcctacaaagtggcagctgaaggcatcaactacgcagacagaaagtggtgttttgatggaattaagaacaaccaaatactggaagaaaatatggaagtggaaatctggacaaaagaaggggaaaggaaaaaattaaaacccagatggttggatgctaggatctattctgacccactagcactaaaagaattcaaggaatttgcagctggaagaaaatctttgaccctgaacctaatcacagaaatgggtaggcttccaactttcatgactcagaaagcaagaaacgcactggacaacctggctgtgctgcatacggctgaggcaggtggaagggcgtacaatcatgctctcagtgaactgccggagaccctggagacactgctcctactgacacttctggcaacagtcacaggaggaatcttcttattcttaatgagcggaaaaggtatagggaagatgaccctgggaatgtgttgcataatcacggctagtatcctcctatggtatgcacagatacaaccacactggatagcagcttcaataatactggagttttttctcatagttttgctcattccagaaccagaaaaacagagaacaccccaagacaaccaattgacctacgttgtcatagccatcctcacagtggtggccgcaaccatggcaaacgagatgggtttcctggaaaaaaccaagaaagacctcggattgggaagcattacaacccaggaatctgagagcaatatcctggacatagatctacgccctgcatcagcatggacgctgtatgccgtagctacaacatttgtcacaccaatgttgagacatagcattgaaaattcctcagtgaatgtctccctaacagccattgctaaccaagctacagtgctaatgggtcttgggaaaggatggccattgtcaaagatggacattggagttcccctccttgccattggatgctattcacaagtcaaccctataactctcacagcagctctccttttattggtagcacattatgccattatagggccaggacttcaagcaaaagcaaccagagaagcccagaaaagagcagcagcaggcatcatgaaaaacccaacagtcgatggaataacagtgattgacctagaaccaataccctatgatccaaaatttgaaaagcagttaggacaagtaatgctcctaatcctctgcgtgactcaagtattaatgatgaggactacatgggctttatgtgaggctctaaccctagcgaccgggcccatctccacactgtgggaaggaaatccagggaggttttggaacactaccattgcagtgtcaatggctaacatctttagggggagctacttggccggagctggacttctcttttccatcatgaaaaacacaacaaacacaagaagaggaactggcaacataggagagacacttggagaaaaatggaaaagtcgattaaacgcactggggaaaagtgaatttcaaatctacaagaaaagtggaatccaggaagtggatagaaccctagcaaaagaaggtatcaaaagaggagaaacggaccaccatgctgtgtcgcgaggttcagcaaaactgagatggttcgtcgagagaaatatggtcacaccggaagggaaggtggtggatctcggttgcggcagagggggctggtcatactattgcgggggactaaagaatgtaagagaagtcaaaggcctaacaaaaggaggaccaggacatgaagaacccatccccatgtcaacatatgggtggaatctagtgcgtctgcaaagtggagttgacgttttcttcaccccgccagaaaagtgtgatacattgttgtgtgacataggggagtcgtcaccaaatcccacgatagaagcaggacgaacactcagagtcctcaacttagtggaaaattggttgaacaataacacccaattttgcataaaggtcctcaacccatatatgccttcagtcatagaaaaaatggaagcattacaaaggaaatatggaggagccttagtgaggaatccactctcacgaaactccacgcatgaaatgtactgggtatctaatgccaccgggaacatagtgtcatcagtgaacatgatttcaaggatgttgattaacagattcacaatgaaacacaagaaagccacttacgagccagatgttgacctaggaagtggaacccgcaacattggaattgaaagtgagataccaaatctagacataataggaaagagaatagagaaaataaaacaagagcatgaaacatcatggcactatgatcaagaccacccatacaaaacgtgggcttaccatggcagctatgaaacaaaacaaactggatcagcatcatctatggtgaacggagtggtcagattgctgacaaaaccttgggacgtcgtccctatggtgacacagatggcaatgacagacacgactccttttggacaacagcgcgttttcaaagagaaagtagacacgagaacccaagaaccgaaggaaggcacaaagaaactgatgaaaattacggcagagtggctttggaaagaactaggaaagaaaaagacacctaggatgtgtaccagagaagaattcacaagaaaagtgagaagcaatgcagccttgggggccatattcactgatgagaacaaatggaaatcggcacgtgaggctgttgaagatggtaggttctgggagctggttgacagggaaagaaatctccatcttgaaggaaagtgtgaaacatgtgtgtacaacatgatgggaaaaagagagaagaaactaggggagttcggcaaggcaaaaggtagcagagccatatggtacatgtggcttggagcacgcttcttagagtttgaagccctaggattcctgaatgaagatcactggttctccagagggaactccctgagtggagtggaaggagaagggctgcacaggctaggctacattttaagagacgtgggcaagaaggaagggggggcaatgtacgccgatgatacagcaggatgggacacaagaatcacactagaagacttaaaaaatgaagaaatggtaacgaaccacatgaaaggagaacacaagaaactagccgaggccatattcaaactaacgtaccaaaacaaggtggtgcgtgtgcaaagaccaacaccaagaggtacagtaatggatatcatatcgagaagagaccaaagaggcagtgggcaagtcggcacctatggccttaataccttcaccaatatggaagcccaattaattagacagatggagggagaaggaatcttcaaaagcattcagcacctgacagccacagaagaaatcgctgtacagaactggctagcaagagtggggcgtgaaaggctatcaagaatggcaatcagtggagatgattgtgttgtaaaacctatagatgacagatttgcaagtgctttaacagctctaaatgacatgggaaaagttagaaaagatatacaacaatgggaaccttcaagaggatggaacgattggacacaagtgcctttctgttcacaccactttcatgagttagtcatgaaagatggtcgcgtgctcgtagtcccatgcagaaaccaagatgaactgattggtagagcccgaatttcccagggagctgggtggtctttgaaagagacggcctgtttgggaaagtcttacgcccaaatgtggactctgatgtacttccacagacgtgacctcagactggcggcaaatgccatctgctcggcagtcccgtcacattgggttccaacaagtcgaacaacctggtccatacacgctaagcatgaatggatgacgacggaagacatgctggcagtctggaacagggtgtggatccaagaaaacccgtggatggaagataaaactccagtggaatcatgggaagaagtcccatacttgggaaaaagagaagaccaatggtgcggctcattgattgggctaacaagcagggctacctgggcaaagaacatccaaacagcaataaatcaagtcagatcccttataggcaatgaggaatacacagactacatgccatccatgaagagatttagaagggaagaggaagaggcaggtgtcctgtggtagaaggcaaaactaacatgaaacaaggctaaaagtcaggtcggattaagccatagtacggaaaaaactatgctacctgtgagccccgtccaaggacgttaaaagaagtcaggccatcacaaaatgccacagcttgagtaaactgtgcagcctgtagctccacctgaggaggtgtaaaaaacctgggaggccacaaaccatggaagctgtacgcatggcgtagtggactagcggttagaggagacccctcccttacaaatcgcagcaaacaacgggggcccaaggtgagatgaagctgtaatctcactggaaggactagaggttagaggagacccccccaaaacaaaaaacagcatattgacgctgggaaagaccagagatcctgctgtctcctcagcatcattccaggcacagaacgccagaaaatggaatggtgctgttgaatcaacaggttct

SEQ ID NO: 11 - DNA, 10708 bp, Dengue virus
  source 1..10708: mol_type = genomic DNA
agttgttagtctacgtggaccgacaagaacagtttcgactcggaagcttgcttaacgtagtgctaacagttttttattagagagcagatctctgatgaacaaccaacggaagaagacgggaaaaccgtctatcaatatgctgaaacgcgtgagaaaccgtgtgtcaactggatcacagttggcgaagagattctcaaaaggactgctgaacggccagggaccaatgaaattggttatggcgttcatagctttcctcagatttctagccattccaccaacagcaggagtcttggctagatggggaaccttcaagaagtcgggggccattaaggtcctgaaaggctttaagaaggagatctcaaacatgctgagcataatcaacaaacggaaaaagacatcgctctgtctcatgatgatattgccagcagcacttgctttccacttgacttcacgagatggagagccgcgcatgattgtggggaagaatgaaagaggaaaatccctactttttaagacagcctctggaattaacatgtgcacactcatagccatggacttgggagagatgtgtgatgacacggtcacttacaaatgcccccatattaccgaagtggaacctgaagacattgactgctggtgcaacctcacatcaacatgggtgacttatggaacgtgcaatcaagccggagagcatagacgcgataagagatcagtggcgttagctccccatgtcggcatgggactggatacacgcacccaaacttggatgtcggctgaaggagcttggaggcaagtcgagaaggtagagacatgggcccttaggcacccagggttcaccatactagccctatttcttgcccattacataggcacttccttgacccagaaggtggttatttttatactgctaatgctggtcaccccatccatgacaatgagatgtgtgggagtaggaaacagagattttgtggaaggactatcaggagctacgtgggttgacgtggtgctcgagcacggggggtgtgtgaccaccatggctaagaacaagcccacgttggatatagagcttcagaagaccgaggccacccaactggcgaccctaaggaagctatgcattgaggggaaaatcaccaacataacaactgactcaagatgtcctacccaaggggaagcggttttgcctgaggagcaggaccaaaactacgtgtgtaagcatacatacgtagacagaggctgggggaacggatgtggtttgtttggtaagggaagcttggtaacatgtgcgaaatttcaatgcctggaaccaatagagggaaaagtggtgcaatatgagaacctcaaatacaccgttatcatcacagtgcacacaggagaccaacaccaggtgggaaatgaaacgcagggagtcacggctgagataacacctcaggcatcaaccactgaagccatcttgcctgaatatggaacccttgggctagaatgctcaccacggacaggtttggacttcaatgaaatgatcttgctaacaatgaagaacaaagcatggatggtacatagacaatggttttttgacctacctctaccatggacatcaggagctacaacggaaacaccaacctggaacaggaaggagcttcttgtgacatttaaaaacgcacatgcgaagaaacaagaagtagtcgttttagggtcacaggagggagctatgcataccgcactaaccggagcgactgagatacagaatagcggagggacatcaatcttcgccggacaccttaagtgtagattgaaaatggacaaacttgagcttaaggggatgtcatacgctatgtgtacgaacacattcgtgctgaaaaaagaggtaagcgaaacgcaacacggaacgatactgattaaggttgagtataagggcgaagacgtcccatgtaagatacctttttcgacagaggacggacagggtaaggcccataacggaagactgattaccgctaacccagtggtgaccaaaaaagaggaaccagtcaatatcgaagccgaacctccattcggagagtcaaacatagtgatagggataggcgataacgcacttaagattaactggtacaaaaaagggtcatcaatcggtaagatgtttgaggcaaccgctaggggggctagacggatggccatactcggagacaccgcatgggacttcggatccgtggggggggtacttaactcactcggtaagatggtgcaccaaattttcggatccgcatataccgctctatttagcggagtgtcatgggtgatgaaaatcggaatcggagttctattgacatggatcggattgaactctaagaatacatctatgtcattttcatgtatcgcaatcggaattattacgctatatctcggagccgtagtgcaagccgacatggggtgtgttataaactggaaaggcaaagaactcaagtgtggaagtggaatcttcgtcaccaacgaggtccatacctggacagagcaatacaaattccaagcagactccccaaaaagattggcgacagccattgcaggcgcttgggagaatggagtgtgcggaattaggtcaacaaccagaatggagaatctcctgtggaagcaaatagccaatgaactgaactacatattgtgggaaaacaatatcaaattaacggttgttgtgggcgatataattggggtcttagagcaagggaaaagaacactaacaccacaacccatggagctaaaatactcatggaaaacgtggggaaaggcaaaaatagtgacagctgaaacacaaaattcttctttcataatagatggaccaaacacaccggagtgtccaagtgcctcaagagcatggaatgtgtgggaggtggaagattacgggttcggagtcttcacaaccaacatatggctgaaactccgagaggtgtatacccaactatgtgaccataggttaatgtcggcagccgtcaaggatgaaagggccgtacatgccgacatgggctattggatagaaagtcaaaagaatggaagttggaagctagaaaaagcatccctcatagaggtgaaaacctgcacatggccaaaatcacataccctttggagtaatggtgtgttagagagtgacatgatcattccaaaaagtctagctggtcctatctcgcaacacaactacaggcccgggtaccacacccagacggcgggaccttggcatttaggaaaattagagctggacttcaactattgtgaaggaacaacagttgtcatcacagaaaactgtgggacaagaggcccatcattgagaacaacaacagtgtcagggaagttaatacacgaatggtgctgccgctcgtgcacacttcctcccctgcgatacatgggagaagacggttgctggtatggcatggaaatcagacccatcagtgagaaagaagaaaacatggtaaagtctttagtctcagcgggaagtggagaggtggacaacttcacaatgggtgtcttgtgtttggcaatcctctttgaagaggtgatgagaggaaaatttgggaagaaacacatgattgcgggggttttcttcacgtttgtactccttctctcagggcaaataacatggagagatatggcgcacacactaataatgattgggtccaatgcatctgacaggatgggaatgggcgtcacctacctagctttaattgcaacatttaaaatccagccatttttggctttgggatttttcctaagaaaactgacatccagagaaaatttattgttaggagttgggctggctatggcaacaacgttacaactgccagaggacattgaacaaatggcaaatggaatcgctctggggctcatggctctcaaactgataacacaatttgaaacataccaactatggacagcattaatctccttaacgtgttcaaatacaatttttacgttgactgttgcctggagaacagccaccctgattttggctggagtttcacttttaccagtgtgccagtcttcgagtatgaggaaaacagactggcttccaatgacagtggcagctatgggagttccacctctaccactttttatttttagcttaaaagacacactcaaaaggagaagctggccactgaatgaaggggtgatggctgttgggcttgtgagcattctggccagttctctccttagaaatgatgtacccatggctggaccattagtggccgggggcttgctgatagcgtgctacgtcataactggcacgtcagcagacctcaccgtagaaaaagcagcagatgtaacatgggaggaagaggctgagcaaacaggagtgtcccacaacttaatgatcacagttgatgatgatggaacaatgagaataaaagatgatgagactgagaatatcttaacagtgcttttgaaaacagcattactaatagtgtcaggaatctttccatactccatacccgcaacattgttggtctggcatacttggcaaaagcaaacccaaagatccggcgttctatgggatgtacccagccctccagagacacagaaagcagaactggaagaaggggtctataggatcaaacagcaaggaatttttgggaaaacccaagtaggggttggagtacagaaagaaggagtctttcacaccatgtggcacgttacaagaggggcagtgttgacatataatgggaaaagactggaaccaaattgggctagcgtgaaaaaagatctgatttcatacggaggaggatggagattgagcgcacaatggcaaaagggggaggaggtgcaggttattgccgtagagcctgggaagaacccaaagaactttcaaaccatgccaggcacttttcagactacaacaggggaaataggagcaattgcactggatttcaagcccggaacttcaggatctcctatcataaacagagagggaaaggtagtgggactgtatggcaatggagtggttacaaagaatggtggctacgtcagcggaatagcgcaaacgaatgcagaaccagatggaccgacaccagaattggaagaagagatgttcaaaaagcgaaatctaaccataatggatcttcatcctgggtcaggaaagacacggaaataccttccagctattgttagagaggcaatcaagagacgtttgagaactctaattctggcaccaacaagggtggttgcagctgagatggaagaagcattgaaagggctcccaataaggtaccaaacaacagcaacaaaatctgaacacacaggaagagagattgttgatctgatgtgccacgcaacgttcacaatgcgtctgctgtcaccagttagggttccaaactataacttgataataatggatgaagcccatttcacagacccagccagtatagctgctagagggtacatatcaactcgtgttggaatgggagaagcagccgcaatattcatgacagcaacgccccctggaacagctgatgcctttccccagagcaacgctccaattcaagatgaagaaagggacataccagaacgctcatggaattcaggcaatgaatggataaccgacttcgctgggaaaacggtgtggtttgtccccagcattaaagccggaaatgacatagcaaattgcctgcggaaaaacgggaaaaaggtcattcaacttagtaggaagacttttgacacagaatatcagaaaaccaaactgaatgattgggactttgtggtgacgactgacatttcagaaatgggggccaatttcaaagcagatagagtgatcgacccaagaagatgtctcaaaccagtgatcctgacagatggaccagagcgggtgatcctggctggaccaatgccagtcaccgcagcgagtgctgcgcaaaggagagggagagttggcaggaacccacaaaaagaaaatgaccagtacatattcacgggccagcctctcaacaatgatgaagaccatgctcactggacagaagcaaaaatgctgctggacaacattaacacaccagaagggatcataccagctctctttgagccagaaagggagaagtcagccgccatagacggtgagtatcgcctgaaaggtgagtccaggaagactttcgtggaactcatgaggaggggtgaccttccagtctggttagcccataaagtagcatcagaagggatcaaatatacagatagaaaatggtgctttgatggacaacgtaataatcaaattttagaagagaacatggatgtggaaatctggacaaaggaaggagaaaagaaaaaattgagacctaggtggcttgatgctcgcacctattcagatcccttagcactcaaggaattcaaggactttgcggctggcaggaagtcaatagcccttgatcttgtgacagaaataggaagagtgccttcacacctagctcatagaacgagaaacgctctggacaatctggtgatgctgcatacgtcagaacatggcggtaaggcctacaggcatgcggtggaggaactaccagagacaatggaaacactcctactcttgggactcatgatcttgttgacaggtggagcaatgcttttcttaatatcaggtaaagggattggaaagacttcaataggactcatttgtgtaattgcttccagcggcatgttgtggatggccgaaatcccactccaatggatcgcgtcggccatagtcctggagttttttatgatggtgttgcttataccagaaccagagaagcagagaaccccccaagacaaccaactcgcatatgtcgtgataggcatacttacactggcagcaataatagcagccaatgaaatgggattgttggaaactacaaagagagatttaggaatgtctaaggagccaggtgttgtttctccaaccagctatttagatgtggacttgcacccagcatcagcctggacattgtacgctgtggccactacagtaataacaccaatgttaagacataccatagagaattccacagcaaatgtgtccttggcagctatagccaaccaggcagtggtcctgatgggtttggacaaaggatggccaatatcaaaaatggacttaggagtacccctgctggcattgggttgctattcacaagtgaacccactgactctaacagcggcagtactcttgctgatcacacattatgccattataggtccaggattgcaggcaaaagccacccgtgaagctcagaaaaggacagctgctggaataatgaagaatccaacagtggatgggataatgacaatagacctagatcctgtaatatatgattcaaaatttgaaaagcaactgggacaggttatgctcctggttttgtgtgcagttcaacttttgttaatgagaacatcatgggccttgtgtgaagctttaaccctagctacaggaccaataacaacactctgggaaggatcacctgggaagttttggaacaccacgatagctgtttccatggcgaacatttttagagggagctatttagcaggagctgggcttgctttctctattatgaaatcagttggaacagggaaaagaggaacaggctcacagggtgaaactttgggagaaaaatggaaaaagaagttaaatcaattatcccggaaagagtttgacctttacaagaaatctggaatcactgaggtggatagaacagaagccaaagaagggttgaaaagaggagaaataacacatcatgccgtgtccagaggtagtgcaaaacttcaatggtttgtggagagaaacatggtcattcccgaaggaagagttatagacttgggctgtggaagaggaggctggtcatattactgtgcaggactgaaaaaagtcacagaagtgcgaggatacacaaaaggcggtccaggacacgaagaaccagtacctatgtccacatatggatggaacatagttaagttaatgagtggaaaggatgtgttttatcttccacctgaaaagtgtgacaccctgttgtgcgacattggagaatcttcaccaagcccaacagtggaagaaagcagaactataagagttttgaagatggttgaaccatggctaaagaacaaccaattttgtattaaagtattgaacccttacatgccaactgtgattgagcacctagaaagactacaaaggaaacatggaggaatgcttgtgagaaatccactttcacgaaactccacgcacgaaatgtactggatatccaatggcacaggtaacattgtcgcttcagtcaacatggtatctagactgctactgaacaggttcacgatgacacacagaagacccaccattgagaaagatgtggatttaggagcaggaactcgacatgttaatgcggaaccagaaacacccaacatggatgtcattggggaaagaataaaaaggatcaaggaggagcataattcaacatggcactacgatgacgaaaacccctacaaaacgtgggcttaccatggatcttatgaagtcaaagccacaggctcagcctcctccatgataaatggagtcgtgaaactcctcactaaaccatgggatgtggtgcccatggtgacacagatggcaatgacagatacaactccatttggccagcagagagtctttaaagagaaagtggacaccaggacacccaggtccatgccaggaacaagaagggttatggggatcacagcggagtggctctggagaaccctgggaaggaataaaaaacccaggttatgcacaagggaagagtttacaaaaaaggtcagaactaacgcagccatgggagctgttttcacagaggagaaccaatgggacagcgcgaaagctgctgttgaggatgaggatttttggaaacttgtggacagagaacgtgaactccacaaactgggcaagtgtggaagctgtgtttacaacatgatgggtaagagagagaagaaacttggagagtttggcaaagcaaaaggcagtagagctatatggtacatgtggttgggagccaggtaccttgagttcgaagcccttggattcttaaatgaagaccactggttctcgcgtgagaactcttacagtggagtggaaggagaaggactgcacaagctaggctatatattaagggacatttccaagatacccggaggagctatgtatgctgatgacacagctggttgggacacaagaataacagaagatgacctgcacaatgaggaaaagatcacacagcaaatggaccctgaacacaggcagttagcgaacgctatatttaagctcacataccaaaacaaagtggtcaaagttcaacgaccgactccaacaggcacggtaatggatatcatatctaggaaagaccaaagaggcagtggacaggtaggaacttatggtctgaatacattcaccaacatggaagcccagttaatcagacaaatggaaggagaaggtgtgctgtcaaaggcagacctcgagaaccctcatctgccagagaagaaaattacacaatggttggaaaccaaaggagtggagaggttaaaaagaatggccataagtggggatgactgcgtggtgaaaccaatcgatgacaggttcgctaatgccctgctcgctctgaacgacatgggaaaggttcggaaagacatacctcaatggcagccatcaaagggatggcatgattggcaacaggttcctttctgctcccaccactttcatgaattgatcatgaaagatggaagaaagttggtggttccctgcagaccccaggacgaactaataggaagggcaagaatctctcaaggagcgggatggagccttagagaaaccgcatgtctggggaaagcctacgctcaaatgtggagtctcatgtattttcacagaagagacctcagactagcatccaacgccatatgttcagcagtaccagtccactgggtccccacaagtagaacgacatggtctattcacgctcaccatcagtggatgaccacagaagacatgcttactgtctggaacagagtgtggatcgaggacaatccatggatggaagacaaaactccagtcacaacctgggaaaatgttccatatctagggaagagagaagaccaatggtgcggatcacttattggtctcacttccagagcaacctgggcccagaacatacccacagcaattcaacaggttagaagccttataggcaatgaagagtttctggactacatgccttcaatgaagagatttaggaaggaggaggagtcggagggagccatttggtaaaacgtaggaagtgaaaaagaggttaactgtcaggccatattaagccacagtacggaagaagctgtgctgcctgtgagccccgtccaaggacgttaaaagaagaagtcaggccccaaagccacggtttgagcaaaccgtgctgcctgtagctccgtcgtggggacgtaaaacctgggaggctgcaaactgtggaagctgtacgcacggtgtagcagactagcggttagaggagacccctcccatgacacaacgcagcagcggggcccgagcactgagggaagctgtacctccttgcaaaggactagaggttagaggagaccccccgcaaataaaaacagcatattgacgctgggagagaccagagatcctgctgtctcctcagcatcattccaggcacagaacgccagaaaatggaatggtgctgttgaatcaacaggttct

SEQ ID NO: 12 - DNA, 10649 bp, Dengue virus
  source 1..10649: mol_type = genomic DNA
agttgttagtctgtgtggaccgacaaggacagttccaaatcggaagcttgcttaacacagttctaacagtttgtttaaatagagagcagatctctggaaaaatgaaccaacgaaaaaaggtggttagaccacctttcaatatgctgaaacgcgagagaaaccgcgtatcaacccctcaagggttggtgaagagattctcaaccggacttttttctgggaaaggacccttacggatggtgctagcattcatcacgtttttgcgagtcctttccatcccaccaacagcagggattctgaagagatggggacagttgaagaaaaataaggccatcaagatactgattggattcaggaaggagataggccgcatgctgaacatcttgaacgggagaaaaaggtcaacgataacattgttgtgcttgattcccaccgtaatggcgtttcacttgtcaacaagagatggcgaacccctcatgatagtggcaaaacatgaaagggggagacctctcttgtttaagacaacagaggggatcaacaaatgcactctcattgccatggacttgggtgaaatgtgtgaggacactgtcacgtataaatgccccctactggtcaataccgaacctgaagacattgattgctggtgcaacctcacgtctacctgggtcatgtatgggacatgcacccagagcggagaacggagacgagagaagcgctcagtagctttgacaccacattcaggaatgggattggaaacaagagctgagacatggatgtcatcggaaggggcttggaagcatgctcagagagtagagagctggatactcagaaacccaggatttgcgctcttggcaggatttatggcttatatgattgggcaaacaggaatccagcgaactgtcttctttgtcctaatgatgctggtcgccccatcctacggaatgcggtgcgtaggagtaggaaacagagactttgtggaaggagtctcaggtggagcatgggtcgacctggtgctagaacatggaggatgcgtcacaaccatggcccagggaaaaccaaccttggattttgaactgactaagacaacagctaaggaagtggctctgttaagaacctattgcattgaagcctcaatatcaaacataactacggcaacaagatgtccaacgcaaggagagccttatctgaaagaggaacaggaccaacagtacatctgccggagagatgtggtagacagaggatggggcaatggctgtggcttgtttggaaaaggaggagttgtgacatgtgcgaagttttcatgttcggggaagataacaggcaatctggtccaaattgagaaccttgaatacacagtggttgtaacagtccacaatggagacacccatgcagtaggaaatgacacatccaatcatggagttacagccacgataactcccaggtcaccatcggtagaagtcaaattgccggactatggagaactaacactcgattgtgaacccaggtctggaattgactttaatgagatgatcctaatgaaaatgaaaaagaaaacatggctcgtgcataagcaatggtttttggatctgcctcttccatggacagcaggagcagacacatcagaggttcactggaattacaaagagagaatggtgacgttcaaggttcctcatgccaagagacaggacgttacagtgttagggtcacaggagggagctatgcatagcgcactagccggagcaaccgaagtcgatagcggagacggaaatcatatgttcgccggacatctgaaatgcaaagtgagaatggagaaattgcggattaagggaatgtcatacactatgtgttccggtaagttttcgattgacaaagagatggccgaaacgcaacacggaacaacagtcgttaaggttaagtacgaaggagccggagctccgtgtaaagtgccaatcgaaattagagacgttaacaaagagaaagtggtcggaagagtgatatctagtacacccctagccgaaaatacgaattccgttacgaatatcgaactcgaacccccctttggagactcatacatagtgataggagtgggtaattccgcactcacgttgcactggttcagaaagggatcatcaatcgggaagatgttcgaatcaacatataggggagcgaaaagaatggctatattgggcgaaaccgcatgggacttcggatcagtcggaggactgtttacgagtctgggtaaggccgtacatcaggtattcggatcagtgtatacaacaatgtttggcggagtgtcatggatgatacggatactgatagggtttctagtgttgtggatcggaacgaactcacgtaatacgtctatggctatgacatgtattgccgtaggggggattacactgtttctgggatttacagtgcaagcagacatgggttgtgtggtgtcatggagtgggagagaattgaagtgtggaagcggaatttttgtggttgacaacgtgcacacttggacagaacagtacaaattccaaccagagtccccagcgagactagcgtctgcaatattaaatgcccacaaagatggggtctgtggaattagatcaaccacgaggctggaaaatgttatgtggaagcaaataaccaatgagctaaactatgttctctgggaaggaggacatgatctcactgtagtggctggggatgtgaaaggggtgttgaccaagggcaagagagcactcacacccccagcgagtgatctgaaatattcatggaagacatgggggaaagcaaaaatcttcacccctgaagcaagaaacagcacatttttaatagacggaccagacacctctgaatgccccaatgaacgaagggcatggaattcttttgaggtggaagactatggatttggcatgttcacgaccaacatatggatgaaattccgagaaggaagttcagaagtgtgtgaccacaggttaatgtcagctgcaattaaagaccagaaagctgtgcatgctgacatgggttattggatagagagctcaaaaaaccagacctggcagatagagagagcatctcttattgaagtgaaaacatgtctgtggcccaagacccatacactgtggagcaatggagtgctggaaagccagatgcttattccaaaatcatatgcaggccctttttcacagcacaattaccgccagggctatgctacgcaaaccgtgggtccatggcacttaggcaaactagagatagactttggagaatgccccggaacaacagtcacaattcaggagaattgtgaccatagaggcccatctttgaggaccaccactgcatctggaaaactagtcacgcaatggtgttgccgctcctgcacgatgccccccttaaggttcttaggagaagatgggtgctggtatgggatggagattaggcccttgagtgaaaaagaagagaacatggtcaaatcacaggtgacggccggacagggcacatcggaaactttttcaatgggtctgttgtgcctgaccttgtttgtggaagaatgcttgaggagaagagtcaccaggaaacacatgatattagctgtggtaatcactctttgtgctatcatcctggggggcctcacatggatggacttgctacgagccctcatcatgttgggggacactatgtctggtagaataggaggacagacccacctagccatcatggcagtgttcaagatgtcaccgggatacgtgctgggtgtgtttttaaggaaactcacttcaagagagacagcactaatggtaataggaatggccatgacaacaacactttcaattccacatgacctcatggaactcattgatggaatatcactaggactaattttgctaaaaatagtaacacagtttgacaacacccaagtgggaaccttagctctttccttgactttcataagatcaacaatgtcattggtcatggcttggaggaccattatggctgtgttgtttgtggtcacactcattcctttgtgcaggacaagctgtcttcaaaaacagtctcattgggtagaaataacagcactcatcctaggagcccaagctctgccagtgtacctaatgactcttatgaaaggagcctcaagaagatcttggcctcttaacgaaggcataatggctgtgggtttggttagtctcttaggaagcgctcttttaaagaatgatgtccctttagctggcccaatggtggcaggaggcttacttctggcggcttacgtaatgagtggcagctcagcagatctgtcactagagaaggccgctaatgtgcagtgggatgaaatggcagacataacaggctcaagtccaatcatagaagtgaagcaagatgaggatggctctttctccatacgggacgtcgaggaaaccaatatgataacccttttggtgaaactggcactgataacggtgtcaggtctctaccccttggcaattccaatcacaatgaccttatggtacatgtggcaagtgaaaacacaaagatcaggagccctgtgggacgtcccttcacccgccgccactcaaaaagccgcactgtctgaaggagtgtacaggatcatgcaaagagggttattcgggaaaactcaggttggagtagggatacacatggaaggtgtatttcacacaatgtggcatgttacaagaggatcggtgatctgccacgagactgggagattggagccatcttgggctgatgtcaggaatgacatgatatcatacggtgggggatggaggcttggagataaatgggacaaagaagaagacgttcaggtcctcgctatagaaccagggaaaaatcccaaacatgtccaaacgaaacctggccttttcaagaccctaactggagaaattggagcagtaacattagatttcaaacccggaacgtctggttctcccattatcaacaggaaaggaaaagtcatcggactctatggaaatggagtggtcaccaaatcaggtgattacgtcagtgccataacacaagccgaaagaattggagagccagattatgaagtggatgaggacatttttcgaaagaaaagactaactataatggacttacaccccggagccggaaagacaaaaagaattcttccatcaatagtgagagaagccttaaaaaggaggctgcgaactttgattttggctcccacgagagtggtggcggccgagatggaagaggccctacgtggactgccaatccgttaccaaaccccagctgtaaaatcagaacacacaggaagagagattgtagacctcatgtgccatgcaaccttcacaacaagacttttgtcatcaaccagagttccaaactacaaccttatagtaatggatgaagcacatttcaccgatccttccagtgtcgcggctagaggatacatttcgaccagggtggaaatgggagaggcagcagccatcttcatgaccgcaacccctcccggagcgacagatccctttccccagagcaacagcccaatagaagacatcgagagagagattccggaaaggtcatggaacacagggttcgactggataacagactaccaagggaaaactgtgtggtttgttcccagcataaaagctggaaatgacattgcaaattgtttgagaaagtcgggaaagaaagttatccagttgagtaggaaaacctttgatacagaatatccaaaaacgaaactcacggactgggactttgtggtcactacagacatatctgaaatgggggctaactttagagctgggagagtgatagaccctagaagatgcctcaagccagttatcctaacagatgggccagagagagtcatcttagcaggtcctattccagtgactccagcaagcgctgctcagagaagagggcgaataggaaggaacccagcacaagaagacgaccaatacgttttctccggagacccactaaaaaatgatgaagaccatgcccactggacagaagcaaagatgctgcttgacaatatctacaccccagaagggatcattccaacattgtttggtccggaaagggaaaaaacccaagctattgatggagagtttcgcctcagaggggaacaaaggaagacttttgtggaattaatgaggagaggagaccttccggtgtggctgagttataaggtagcttctgctggcatttcttacaaagatcgggaatggtgctttactggggaaagaaataaccaaattttagaagaaaacatggaggttgaaatttggactagagagggagaaaagaaaaaactgaggccaaaatggttagatgcacgtgtatacgctgaccccatggctttgaaggatttcaaggagtttgccagtggaaggaagagtataactctcgacatcctaacagagatcgccagtttgccaacttacctttcctctagggccaagctcgcccttgacaacatagttatgctccacacaacagaaagaggagggagggcctatcaacatgccctgaacgaacttccggagtcactggaaacactcatgcttgtagccttactaggagctatgacagcaggtatcttcctgtttttcatgcaagggaaaggaatagggaaattgtcaatgggtttgataaccattgcggtggctagtggcttgctctgggtagcagaaattcaaccccagtggatagcggcctcaatcatactggagttttttctcatggtactgttgataccagaaccagaaaaacaaaggaccccacaagacaatcaattgatctacgtcatattgaccattctcaccattattggtctaatagcagccaacgagatggggctgatagaaaaaacaaaaacggattttgggttttaccaggtaaaaacagaaaccaccatcctcgatgtggacctgagaccagcttcagcatggacgctctatgcggtagccaccacaattctgactcccatgctgagacacaccatagaaaatacgtcggccaacctatctttagcagccatcgccaaccaggcagccgtcctaatggggcttggaaaaggatggccactccacagaatggacctcggtgtgccgctgttagcaatgggatgctattctcaagtgaacccaacaaccttgacagcatccttagtcatgcttttagtccattatgcaataataggcccaggattgcaggcaaaagccacaagagaggcccagaaaaggacagctgctggaatcatgaaaaatcccacagtggacgggataacagtgatagatctagaaccaatatcctatgacccaaaatttgaaaagcaattagggcaggtcatgttactcgtcttgtgtgctggacaactactcttgatgagaacaacatgggctttctgtgaagttttgactttggccacaggaccaatcttgaccttgtgggagggcaacccgggaaggttttggaacacgaccatagccgtatctaccgccaacattttcaggggaagttatttggcaggagctggactggctttttcactcataaagaatgcacaaacccccaggaggggaactgggaccacaggagagacactgggagagaagtggaagagacagctaaactcattagacaggaaagagtttgaagagtataaaagaagtggaatactagaagtggacaggactgaagccaagtccgccctgaaagatgggtctaaaatcaagcatgcagtatctagagggtccagtaagatcagatggattgttgagagagggatggtaaagccaaaggggaaagttgtagatcttggctgtgggagaggaggatggtcttattacatggcgacactcaagaacgtgactgaagtgaaagggtatacaaaaggaggtccaggacatgaagaaccgattcccatggctacttatggctggaatttggtcaaactccattcaggggttgacgtgttctacaaacccacagagcaagtggacaccctgctctgtgatattggggagtcatcttctaatccaacaatagaggaaggaagaacattaagagttttgaagatggtggagccatggctctcttcaaaacctgaattctgcatcaaagtcctcaacccctacatgccaacagtcatagaggagctggagaaactgcagagaaaacacggtgggaaccttgtcagatgcccgctgtccaggaactccacccatgagatgtattgggtgtcaggagcgtcgggaaatattgtgagctctgtgaacacaacatcaaagatgttgttgaacaggttcacaacaaggcataggaaacccacttatgagaaggacgtagatcttggggcaggaacgagaagtgtctctactgaaacagaaaaaccagacatgacaatcattgggagaaggcttcagcgattgcaagaggagcacaaagaaacatggcattatgatcaggaaaacccatacagaacctgggcgtatcatggaagctatgaagctccttcgacaggctctgcatcctccatggtgaacggggtggtgaaactgctaacaaaaccctgggatgtgattccaatggtgactcagttagccatgacagatacaaccccttttgggcaacaaagagtgttcaaagagaaggtggataccagaacgccgcaaccaaaaccaggcacacgaatggttatgaccacgacagccaattggctatgggccctccttggaaagaagaaaaatcccagactgtgtacaagggaagagttcatctcaaaagttagatcaaacgcagccataggcgcagtctttcaggaagaacaaggatggacatcagccagtgaagctgtgaatgacagccggttttgggaactggttgacaaagaaagggcccttcaccaggaagggaaatgtgaatcgtgtgtctataacatgatgggaaaacgtgagaaaaagttaggagagtttggcagagccaagggaagccgagcaatctggtacatgtggctgggagcgcggtttctggaatttgaagccctgggttttttgaatgaagatcactggtttggcagagaaaattcatggagtggagtggaaggggaaggtctgcacagattgggatacatcctggaggagatagacaagaaggatggagacctaatgtatgctgatgacacagcaggttgggacacaagaatcactgaggatgaccttcaaaatgaggaactgatcacggaacagatggctccccaccacaagatcctagccaaagccattttcaaactaacctatcaaaacaaagtggtgaaagtcctcagacccacaccgagaggagcggtgatggatatcatatccaggaaagaccaaagaggtagtggacaagttggaacatatggtttgaacacattcaccaacatggaagttcaactcatccgccaaatggaagctgaaggagtcatcacacaagatgacatgcagaacccaaaagggttgaaagaaagagttgagaaatggctgagagagtgtggtgtcgacaggttaaagaggatggcaatcagtggagacgattgcgtggtgaagcccctagatgagaggtttggcacttccctcctcttcttgaacgacatgggaaaggtgaggaaagacattccgcagtgggaaccatctaagggatggaaaaactggcaagaggttcctttttgctcccatcactttcacaagatctttatgaaggatggccgctcactagttgttccatgtagaaaccaggatgaactgatagggagagccagaatctcgcagggggctggatggagcttaagagaaacagcctgcctgggcaaagcttacgcccagatgtggtcgcttatgtacttccacagaagggatctgcgtttagcctccatggccatatgctcagcagttccaacggaatggtttccaacaagcagaacaacatggtcaatccatgctcatcaccaatggatgaccactgaagacatgctcaaagtgtggaacagagtgtggatagaagacaaccccaatatgattgacaagactccagtccattcgtgggaagatataccttacctagggaaaagagaggatttgtggtgtggatccctgattggactttcttctagagccacctgggcgaagaacattcacacggccataactcaggtcaggaacttgatcggaaaagaggaatacgtggattacatgccagtaatgaaaagatacagtgctccttcagagagtgaaggagttctgtaattaccaacaacaaacaccaaaggctattgaagtcaggccacttgtgccacggtttgagcaaaccgtgctgcctgtagctccgccaataatgggaggcgtaataatccctagggaggccatgcgccacggaagctgtacgcgtggcatattggactagcggttagaggagacccctcccatcactgacaaaacgcagcaaaagggggcccgaagccaggaggaagctgtactcctggtggaaggactagaggttagaggagacccccccaacacaaaaacagcatattgacgctgggaaagaccagagatcctgctgtctctacaacatcaatccaggcacagagcgccgcaagatggattggtgttgttgatccaacaggttct